European Patent Application EP 4 484 563 A1, published January 1, 2025. Title: Viral Vector and Producer Cell. Applicant: EsoBiotec. Application EM, filed July 1, 2024. The sequence listing filed with the application follows.

SEQUENCE LISTING (204 sequences)

SEQ ID NO: 1 - protein, 120 aa, synthetic construct
QVQLVESGGGLVQAGGSLRLSCALSGRVWGSYAMGWFRQAPGKEREFVAAISRSGGTTYYADAVKGRFTISRDNGKNTVYLQMNSLKPEDTALYYCATHTNQGPAGFGSWGQGTQVTVSS

SEQ ID NO: 2 - protein, 119 aa, synthetic construct
QVQLVESGGGLVQPGGSLRLSCAASGSISSIYVMGWYRQAPGKQRELVADITRTGTINYLKSVMGRFAISRDNAKSTVYLQMNSLKPEDTAVYYCRVVASAAPGRFGSWGQGTQVTVSS

SEQ ID NO: 3 - protein, 118 aa, synthetic construct
QVQLVESGGGLAQPGGSLRLSCAASGSISSIYVMGWYRQAPGKQRELVADITRTGTINYLKSVMGRFAISRDNAKSTVYLQMNSLKPEDTAVYYCNIRLGYSLGDNYWGQGTQVTVSS

SEQ ID NO: 4 - protein, 118 aa, synthetic construct
QLQLVESGGGLVQPGGSLRLSCAASGSISSIYVMGWYRQAPGKQRELVADITRTGTINYLKSVMGRFAISRDNAKSTVYLQMNSLKPEDTAVYYCNIRLGYSLGDNYWGQGTQVTVSS

SEQ ID NO: 5 - protein, 206 aa, synthetic construct
QVQLQESGGGSVQPGGSLRLSCAASGFTFDDYAMSWVRQVPGKGLEWVSTINWNGGSAEYAEPVKGRFTISRDNAKNTVYLQMNSLKLEDTAVYYCAKDADLVWYNLSTGQGTQVTVSSAAAYPYDVPDYGSGIRGCRSTSGGGGSGGGGSGGGGSNAVGQDTQEVIVVPHSLPFKVVVISAILALVVLTIISLIILIMLWQKKPR

SEQ ID NO: 6 - protein, 198 aa, synthetic construct
EVQLVESGGGLVQPGGSLRLSCAASGFTFDDYVIGWFRQAPGKGREGVACIRIFDRHTYYADSVKGRFTISSDNSKNTVYLQMNSLRAEDTATYYCAAGSFFGCTRPEGDMDYFGQGTLVQVQSGIRGCRSTSGGGGSGGGGSGGGGSNAVGQDTQEVIVVPHSLPFKVVVISAILALVVLTIISLIILIMLWQKKPR

SEQ ID NO: 7 - protein, 204 aa, synthetic construct
EVQLVESGGGLVQPGGSLRLSCAASGFTFDDYAIGWFRQAPGKGREGVACIRIFDRHTYYADSVKGRFTISSDNSKNTVYLQMNSLRAEDTATYYCAAGSFWGCTRPEGDMDYFGQGTLVQVQSGASAKPTTTPAPRPPTPAPTIASQPLSLRPEAARPAAGGAVHTRGLDFAKVVVISAILALVVLTIISLIILIMLWQKKPR

SEQ ID NO: 8 - protein, 204 aa, synthetic construct
EVQLVESGGGLVQPGGSLRLSCAASGFTFEDYAIGWFRQAPGKGREGVACIRIFDRHTYYADSVKGRFTISSDNSKNTVYLQMNSLRAEDTATYYCAAGSFFGCTRPEGDMDYFGQGTLVQVQSGASAKPTTTPAPRPPTPAPTIASQPLSLRPEAARPAAGGAVHTRGLDFAKVVVISAILALVVLTIISLIILIMLWQKKPR

SEQ ID NO: 9 - protein, 117 aa, synthetic construct
EVQLVESGGGLVQPGGSLRLSCAASGDVHKINILGWYRQAPAKEREMVAHITIGDATDYADSAKGRFTISRDEAKNMVYLQMNSLKPEDTAVYFCRAYSRIYPYNYWGQGTLVTVSS

SEQ ID NO: 10 - protein, 241 aa, synthetic construct
EVQLQQSGPELVKPGASVKMSCKASGYKFTSYVMHWVKQKPGQGLEWIGYINPYNDVTKYNEKFKGKATLTSDKSSSTAYMELSSLTSEDSAVHYCARGSYYDYDGFVYWGQGTLVTVSAGGGGSGGGGSGGGGSQIVLTQSPAIMSASPGEKVTMTCSATSSVSYMHWYQQKSGTSPKRWIYDTSKLASGVPARFSGSGSGTSYSLTISSMEAEDAATYYCQQWSSNPLTFGAGTKLELK

SEQ ID NO: 11 - DNA, 898 bp, synthetic construct
  source 1..898: mol_type = other DNA
aaataaacaaggagatagggtgtttattttatggacaagtttcttttgtaacttgtaactcccttgaaagtcagccagagtatgtctcaaaccaaagtcaagatagtgagcaagaagtgttgcacttatgaagggaggtgagtgagcaatgcatgtggtttccaaccgttaatgctagagttatcactttctgttatcaagtggcttcagctatgcaaggaaaccaaacaggggaagttttctcaagcaggttgaaagcaggttccaagaaagccctttgaagtcattaatctgggtgtaatggggctcagctacagagaagcgtatccagaggaaatgtggggttcctgcagtcagctggggcaccgaaaagacccagactttagaaccagataaaggctgagttcgaacctctggttcttttgtgatgtggtgaccttgggcaaattaatgtgtgaacctcagtttcctcaactataaaatgtaatgaacaatacctaccacttactatagaaatctagctgctacggcttgcgctatggggccgacggcttctctcaaggggcttcgagatgtggcagtgtttaggttgtgtgtaaatgtggttgcattgtcaatagggacgctaaagttcaggccaccttttccatattctctgccagctccctgctcagagatagagcaatttacaccgcttccttcctaccctacccctagcccacccccactctgaaaatttcccaccatcaacggcagaaagcagagaagcagacatcttctagttcctcccccactctcctctttccggtacctgtgagtcagctaggggagggcagctctcacccaggctgatagttcggtgacctggctttatctactggatgagttccgctgggag

SEQ ID NO: 12 - DNA, 853 bp, synthetic construct
  source 1..853: mol_type = other DNA
gttctgagcccagtgctggctgccgggctgtttatctctgagtcacatcagcaccaagccacagcagccacctgccctagctccatctcttacagtcacaacaggatgtggtttgacatttactgggtcctgcatctggggtgcctgtgaaagttgctccctccacccacccaccttcagagcatcatgagaaccacactcaccgcatccggcacccaaccccctcctatgctgctctttctacctgggcccctggttagcatcctggcagtagaggcattcatgcttacccacgggctggtcaacaaagaggtgctgacctgagagtagggcacataacctcagccactggggtacacttaccacccccgcccccgtgtagctccctcccctatcctgaaatctcccttagcacactaagtattctaggttaaacagcccagatgttcagggagttcattcgccaagaaatctagctgctacggcttgcgctatggggccgacggcttctctcaaggggcttcgagatgtggcagtgtttaggttgtgtgtaaatgtggttgcattgtcaatagggacgctaaagttcaggccaccttttccatattctctgccagctccctgctcagagatagagcaatttacaccgcttccttcctaccctacccctagcccacccccactctgaaaatttcccaccatcaacggcagaaagcagagaagcagacatcttctagttcctcccccactctcctctttccggtacctgtgagtcagctaggggagggcagctctcacccaggctgatagttcggtgacctggctttatctactggatgagttccgctgggag

SEQ ID NO: 13 - DNA, 1016 bp, synthetic construct
  source 1..1016: mol_type = other DNA
ggtgggaagtaatgagatgtaaatcggggtcttttaggtaatagctgacaactggggtaggaatgggggttctgagcccagtgctggctgccgggctgtttatctctgagtcacatcagcaccaagccacagcagccacctgccctagctccatctcttacagtcacaacaggatgtggtttgacatttactgggtcctgcatctggggtgcctgtgaaagttgctccctccacccacccaccttcagagcatcatgagaaccacactcaccgcatccggcacccaaccccctcctatgctgctctttctacctgggcccctggttagcatcctggcagtagaaatagaaaaataaacaaggagatagggtgtttattttatggacaagtttcttttgtaacttgtaactcccttgaaagtcagccagagtatgtctcaaaccaaagtcaagatagtgagcaagaagtgttgcacttatgaagggaggtgagtgagcaatgcatgtggtttccaaccgttaatgctagagttatcactttctgttatcaagtggcttcagctatgcaaggaaaccaaacaggggaagttttctcaagcaggttgaaagcaggttccaagaaagccctttagaaatctagctgctacggcttgcgctatggggccgacggcttctctcaaggggcttcgagatgtggcagtgtttaggttgtgtgtaaatgtggttgcattgtcaatagggacgctaaagttcaggccaccttttccatattctctgccagctccctgctcagagatagagcaatttacaccgcttccttcctaccctacccctagcccacccccactctgaaaatttcccaccatcaacggcagaaagcagagaagcagacatcttctagttcctcccccactctcctctttccggtacctgtgagtcagctaggggagggcagctctcacccaggctgatagttcggtgacctggctttatctactggatgagttccgctgggag

SEQ ID NO: 14 - DNA, 1016 bp, synthetic construct
  source 1..1016: mol_type = other DNA
aaataaacaaggagatagggtgtttattttatggacaagtttcttttgtaacttgtaactcccttgaaagtcagccagagtatgtctcaaaccaaagtcaagatagtgagcaagaagtgttgcacttatgaagggaggtgagtgagcaatgcatgtggtttccaaccgttaatgctagagttatcactttctgttatcaagtggcttcagctatgcaaggaaaccaaacaggggaagttttctcaagcaggttgaaagcaggttccaagaaagccctttggtgggaagtaatgagatgtaaatcggggtcttttaggtaatagctgacaactggggtaggaatgggggttctgagcccagtgctggctgccgggctgtttatctctgagtcacatcagcaccaagccacagcagccacctgccctagctccatctcttacagtcacaacaggatgtggtttgacatttactgggtcctgcatctggggtgcctgtgaaagttgctccctccacccacccaccttcagagcatcatgagaaccacactcaccgcatccggcacccaaccccctcctatgctgctctttctacctgggcccctggttagcatcctggcagtagaaatagaaagaaatctagctgctacggcttgcgctatggggccgacggcttctctcaaggggcttcgagatgtggcagtgtttaggttgtgtgtaaatgtggttgcattgtcaatagggacgctaaagttcaggccaccttttccatattctctgccagctccctgctcagagatagagcaatttacaccgcttccttcctaccctacccctagcccacccccactctgaaaatttcccaccatcaacggcagaaagcagagaagcagacatcttctagttcctcccccactctcctctttccggtacctgtgagtcagctaggggagggcagctctcacccaggctgatagttcggtgacctggctttatctactggatgagttccgctgggag

SEQ ID NO: 15 - DNA, 928 bp, synthetic construct
  source 1..928: mol_type = other DNA
ggcattcatgcttacccacgggctggtcaacaaagaggtgctgacctgagagtagggcacataacctcagccactggggtacacttaccacccccgcccccgtgtagctccctcccctatcctgaaatctcccttagcacactaagtattctaggttaaacagcccagatgttcagggagttcattcgccaggtgggaagtaatgagatgtaaatcggggtcttttaggtaatagctgacaactggggtaggaatgggggttctgagcccagtgctggctgccgggctgtttatctctgagtcacatcagcaccaagccacagcagccacctgccctagctccatctcttacagtcacaacaggatgtggtttgacatttactgggtcctgcatctggggtgcctgtgaaagttgctccctccacccacccaccttcagagcatcatgagaaccacactcaccgcatccggcacccaaccccctcctatgctgctctttctacctgggcccctggttagcatcctggcagtagaaatagaaagaaatctagctgctacggcttgcgctatggggccgacggcttctctcaaggggcttcgagatgtggcagtgtttaggttgtgtgtaaatgtggttgcattgtcaatagggacgctaaagttcaggccaccttttccatattctctgccagctccctgctcagagatagagcaatttacaccgcttccttcctaccctacccctagcccacccccactctgaaaatttcccaccatcaacggcagaaagcagagaagcagacatcttctagttcctcccccactctcctctttccggtacctgtgagtcagctaggggagggcagctctcacccaggctgatagttcggtgacctggctttatctactggatgagttccgctgggag

SEQ ID NO: 16 - DNA, 860 bp, synthetic construct
  source 1..860: mol_type = other DNA
ggcattcatgcttacccacgggctggtcaacaaagaggtgctgacctgagagtagggcacataacctcagccactggggtacacttaccacccccgcccccgtgtagctccctcccctatcctgaaatctcccttagcacactaagtattctaggttaaacagcccagatgttcagggagttcattcgccaaaataaacaaggagatagggtgtttattttatggacaagtttcttttgtaacttgtaactcccttgaaagtcagccagagtatgtctcaaaccaaagtcaagatagtgagcaagaagtgttgcacttatgaagggaggtgagtgagcaatgcatgtggtttccaaccgttaatgctagagttatcactttctgttatcaagtggcttcagctatgcaaggaaaccaaacaggggaagttttctcaagcaggttgaaagcaggttccaagaaagccctttgaaagaaatctagctgctacggcttgcgctatggggccgacggcttctctcaaggggcttcgagatgtggcagtgtttaggttgtgtgtaaatgtggttgcattgtcaatagggacgctaaagttcaggccaccttttccatattctctgccagctccctgctcagagatagagcaatttacaccgcttccttcctaccctacccctagcccacccccactctgaaaatttcccaccatcaacggcagaaagcagagaagcagacatcttctagttcctcccccactctcctctttccggtacctgtgagtcagctaggggagggcagctctcacccaggctgatagttcggtgacctggctttatctactggatgagttccgctgggag

SEQ ID NO: 17 - DNA, 969 bp, synthetic construct
  source 1..969: mol_type = other DNA
ttagtggtatcaactggccaaaagatgatgttgagtttagtgttcttgagatgagatgaggcaataaatgaagaggaaggacagtggtaaagaacgcactagaaccgtaggcattggcatttgaggtttcagaatgactaatattttagatgaatttgtttgacattgaatgttcatgtgcttctgagcagggtttcaatttgagtaaccgttgcaataacatggggcagctgttttgctctttgtcttcatgacaactgtacttaagctaacagccctgaaacatgagattaggctgggcagaaataaacaaggagatagggtgtttattttatggacaagtttcttttgtaacttgtaactcccttgaaagtcagccagagtatgtctcaaaccaaagtcaagatagtgagcaagaagtgttgcacttatgaagggaggtgagtgagcaatgcatgtggtttccaaccgttaatgctagagttatcactttctgttatcaagtggcttcagctatgcaaggaaaccaaacaggggaagttttctcaagcaggttgaaagcaggttccaagaaagccctttagaaatctagctgctacggcttgcgctatggggccgacggcttctctcaaggggcttcgagatgtggcagtgtttaggttgtgtgtaaatgtggttgcattgtcaatagggacgctaaagttcaggccaccttttccatattctctgccagctccctgctcagagatagagcaatttacaccgcttccttcctaccctacccctagcccacccccactctgaaaatttcccaccatcaacggcagaaagcagagaagcagacatcttctagttcctcccccactctcctctttccggtacctgtgagtcagctaggggagggcagctctcacccaggctgatagttcggtgacctggctttatctactggatgagttccgctgggag

SEQ ID NO: 18 - DNA, 969 bp, synthetic construct
  source 1..969: mol_type = other DNA
aaataaacaaggagatagggtgtttattttatggacaagtttcttttgtaacttgtaactcccttgaaagtcagccagagtatgtctcaaaccaaagtcaagatagtgagcaagaagtgttgcacttatgaagggaggtgagtgagcaatgcatgtggtttccaaccgttaatgctagagttatcactttctgttatcaagtggcttcagctatgcaaggaaaccaaacaggggaagttttctcaagcaggttgaaagcaggttccaagaaagccctttttagtggtatcaactggccaaaagatgatgttgagtttagtgttcttgagatgagatgaggcaataaatgaagaggaaggacagtggtaaagaacgcactagaaccgtaggcattggcatttgaggtttcagaatgactaatattttagatgaatttgtttgacattgaatgttcatgtgcttctgagcagggtttcaatttgagtaaccgttgcaataacatggggcagctgttttgctctttgtcttcatgacaactgtacttaagctaacagccctgaaacatgagattaggctgggcagagaaatctagctgctacggcttgcgctatggggccgacggcttctctcaaggggcttcgagatgtggcagtgtttaggttgtgtgtaaatgtggttgcattgtcaatagggacgctaaagttcaggccaccttttccatattctctgccagctccctgctcagagatagagcaatttacaccgcttccttcctaccctacccctagcccacccccactctgaaaatttcccaccatcaacggcagaaagcagagaagcagacatcttctagttcctcccccactctcctctttccggtacctgtgagtcagctaggggagggcagctctcacccaggctgatagttcggtgacctggctttatctactggatgagttccgctgggag

SEQ ID NO: 19 - DNA, 1040 bp, synthetic construct
  source 1..1040: mol_type = other DNA
ttagtggtatcaactggccaaaagatgatgttgagtttagtgttcttgagatgagatgaggcaataaatgaagaggaaggacagtggtaaagaacgcactagaaccgtaggcattggcatttgaggtttcagaatgactaatattttagatgaatttgtttgacattgaatgttcatgtgcttctgagcagggtttcaatttgagtaaccgttgcaataacatggggcagctgttttgctctttgtcttcatgacaactgtacttaagctaacagccctgaaacatgagattaggctgggcagggtgggaagtaatgagatgtaaatcggggtcttttaggtaatagctgacaactggggtaggaatgggggttctgagcccagtgctggctgccgggctgtttatctctgagtcacatcagcaccaagccacagcagccacctgccctagctccatctcttacagtcacaacaggatgtggtttgacatttactgggtcctgcatctggggtgcctgtgaaagttgctccctccacccacccaccttcagagcatcatgagaaccacactcaccgcatccggcacccaaccccctcctatgctgctctttctacctgggcccctggttagcatcctggcagtagaaatagaaagaaatctagctgctacggcttgcgctatggggccgacggcttctctcaaggggcttcgagatgtggcagtgtttaggttgtgtgtaaatgtggttgcattgtcaatagggacgctaaagttcaggccaccttttccatattctctgccagctccctgctcagagatagagcaatttacaccgcttccttcctaccctacccctagcccacccccactctgaaaatttcccaccatcaacggcagaaagcagagaagcagacatcttctagttcctcccccactctcctctttccggtacctgtgagtcagctaggggagggcagctctcacccaggctgatagttcggtgacctggctttatctactggatgagttccgctgggag

SEQ ID NO: 20 - DNA, 1040 bp, synthetic construct
  source 1..1040: mol_type = other DNA
ggtgggaagtaatgagatgtaaatcggggtcttttaggtaatagctgacaactggggtaggaatgggggttctgagcccagtgctggctgccgggctgtttatctctgagtcacatcagcaccaagccacagcagccacctgccctagctccatctcttacagtcacaacaggatgtggtttgacatttactgggtcctgcatctggggtgcctgtgaaagttgctccctccacccacccaccttcagagcatcatgagaaccacactcaccgcatccggcacccaaccccctcctatgctgctctttctacctgggcccctggttagcatcctggcagtagaaatagaattagtggtatcaactggccaaaagatgatgttgagtttagtgttcttgagatgagatgaggcaataaatgaagaggaaggacagtggtaaagaacgcactagaaccgtaggcattggcatttgaggtttcagaatgactaatattttagatgaatttgtttgacattgaatgttcatgtgcttctgagcagggtttcaatttgagtaaccgttgcaataacatggggcagctgttttgctctttgtcttcatgacaactgtacttaagctaacagccctgaaacatgagattaggctgggcagagaaatctagctgctacggcttgcgctatggggccgacggcttctctcaaggggcttcgagatgtggcagtgtttaggttgtgtgtaaatgtggttgcattgtcaatagggacgctaaagttcaggccaccttttccatattctctgccagctccctgctcagagatagagcaatttacaccgcttccttcctaccctacccctagcccacccccactctgaaaatttcccaccatcaacggcagaaagcagagaagcagacatcttctagttcctcccccactctcctctttccggtacctgtgagtcagctaggggagggcagctctcacccaggctgatagttcggtgacctggctttatctactggatgagttccgctgggag

SEQ ID NO: 21 - protein, 19 aa, synthetic construct
AVGQDTQEVIVVPHSLPFK

SEQ ID NO: 22 - protein, 6 aa, synthetic construct
GAPGAS

SEQ ID NO: 23 - protein, 17 aa, synthetic construct
GAPGSGGGGSGGGGSAS

SEQ ID NO: 24 - protein, 39 aa, synthetic construct
ASGGGGSGELAAIKQELAAIKKELAAIKWELAAIKQGAG

SEQ ID NO: 25 - protein, 14 aa, synthetic construct
ASESKYGPPCPPCP

SEQ ID NO: 26 - protein, 50 aa, synthetic construct
PAKPTTTPAPRPPTPAPTIASQPLSLRPEACRPAAGGAVHTRGLDFACDI

SEQ ID NO: 27 - protein, 30 aa, synthetic construct
VVVISAILALVVLTIISLIILIMLWQKKPR

SEQ ID NO: 28 - protein, 42 aa, synthetic construct
WAITLISVNGIFVICCLTYCFAPRCRERRRNERLRRESVRPV

SEQ ID NO: 29 - protein, 326 aa, synthetic construct
METDTLLLWVLLLWVPGSTGDQVQLQQSGAELARPGASVKMSCKASGYTFTRYTMHWVKQRPGQGLEWIGYINPSRGYTNYNQKFKDKATLTTDKSSSTAYMQLSSLTSEDSAVYYCARYYDDHYCLDYWGQGTTLTVSSGGGGSGGGGSGGGGSQIVLTQSPAIMSASPGEKVTMTCSASSSVSYMNWYQQKSGTSPKRWIYDTSKLASGVPAHFRGSGSGTSYSLTISGMEAEDAATYYCQQWSSNPFTFGSGTKLEINRGGGGSGGGGSGGGGSAVGQDTQEVIVVPHSLPFKVVVISAILALVVLTIISLIILIMLWQKKPR

SEQ ID NO: 30 - protein, 274 aa, synthetic construct
METLLGLLILWLQLQWVSSKQEVTQIPAALSVPEGENLVLNCSFTDSAIYNLQWFRQDPGKGLTSLLLIQSSQREQTSGRLNASLDKSSGRSTLYIAASQPGDSATYLCAVRPLYGGSYIPTFGRGTSLIVHPYIQNPDPAVYQLRDSKSSDKSVCLFTDFDSQTNVSQSKDSDVYITDKCVLDMRSMDFKSNSAVAWSNKSDFACANAFNNSIIPEDTFFPSPESSCDVKLVEKSFETDTNLNFQNLSVIGFRILLLKVAGFNLLMTLRLWSS

SEQ ID NO: 31 - protein, 311 aa, synthetic construct
MSIGLLCCAALSLLWAGPVNAGVTQTPKFQVLKTGQSMTLQCAQDMNHEYMSWYRQDPGMGLRLIHYSVGAGITDQGEVPNGYNVSRSTTEDFPLRLLSAAPSQTSVYFCASSYVGNTGELFFGEGSRLTVLEDLKNVFPPEVAVFEPSEAEISHTQKATLVCLATGFYPDHVELSWWVNGKEVHSGVCTDPQPLKEQPALNDSRYCLSSRLRVSATFWQNPRNHFRCQVQFYGLSENDEWTQDRAKPVTQIVSAEAWGRADCGFTSESYQQGVLSATILYEILLGKATLYAVLVSALVLMAMVKRKDSRG

SEQ ID NO: 32 - protein, 491 aa, synthetic construct
MGQIVTFFQEVPHVIEEVMNIVLIALSVLAVLKGLYNFATCGLVGLVTFLLLCGRSCTTSLYKGVYELQTLELNMETLNMTMPLSCTKNNSHHYIMVGNETGLELTLTNTSIINHKFCNLSDAHKKNLYDHALMSIISTFHLSIPNFNQAEAMSCDFNGGKISVQYNLSHSYAGDAANHCGTVANGVLQTFMRMAWGGSYIALDSGRGNWDCIMTSYQYLIIQNTTWEDHCQFSRPSPIGYLGLLSQRTRDIYISRRLLGTFTWTLSDSEGKDTPGGYCLTRWMLIEAELKCFGNTAVAKCNEKHDEEFCDMLRLFDFNKQAIQRLKAEAQMSIQLINKAVNALINDQLIMKNHLRDIMGIPYCNYSKYWYLNHTTTGRTSLPKCWLVSNGSYLNETHFSDDIEQQADNMITEMLQKEYMERQGKTPLGLVDLFVFSTSFYLISIFLHLVKIPTHRHIVGKSCPKPHRLNHMGICSCGLYKQPGVPVKWKR

SEQ ID NO: 33 - protein, 523 aa, synthetic construct
MWIITALICSFSINPTCLYPHGHEDSPTVRHGISRVLSGDAERNDDEHYHSPPLVLPLQNERTWKPANLSSLKCPEASHLGPDEHRVMEKWLVHRPKSSVLTKVEGSLCHKSRWLTRCEYTWYFSKTVSRKIEPMPPTKQECEEAIKRKEEGLLESLGFPPPACYWARTNDEENVQVDVTDHPMTYDPYSDGVVDNILVGGKCNQRECETVHDSTIWLETQKEKRPSQCEMDVEEQLELVSGIKRVGGSKSKAQRSVFVVGTNYPFMDATGACRLKYCSKSGMLLSNGLWFHITRKISPESNENSKFWLTLSDCSSDKQVGVLGEEYEIGKLQATMEDIMWDLDCFRTLEDLSHHKKVSMLDLFRLSRLTPGTGPAYKLVKGNLMVKEVQYVKAQRDQGELANPLCVAFMTESKNADRCIRYDEYDKEGPYKGQVMNGILINEGMVVFPHERFHLRQWDPEFIIKHEIKQVHHPVLGNYSSQIHDSLHESLIKDHSANLGDVMGNWVQVATSKFSWFFKEIEK

SEQ ID NO: 34 - protein, 201 aa, synthetic construct
METDTLLLWVLLLWVPGSTGDEVQLVESGGGLVQPGGSLRLSCAASGDVHKINILGWYRQAPAKEREMVAHITIGDATDYADSAKGRFTISRDEAKNMVYLQMNSLKPEDTAVYFCRAYSRIYPYNYWGQGTLVTVSSASESKYGPPCPPCPAVGQDTQEVIVVPHSLPFKVVVISAILALVVLTIISLIILIMLWQKKPR

SEQ ID NO: 35 - protein, 486 aa, synthetic construct
MALPVTALLLPLALLLHAARPQVKLEESGGGLVQAGRSLRLSCAASEHTFSSHVMGWFRQAPGKERESVAVIGWRDISTSYADSVKGRFTISRDNAKKTLYLQMNSLKPEDTAVYYCAARRIDAADFDSWGQGTQVTVSSGGGGSEVQLVESGGGLVQAGGSLRLSCAASGRTFTMGWFRQAPGKEREFVAAISLSPTLAYYAESVKGRFTISRDNAKNTVVLQMNSLKPEDTALYYCAADRKSVMSIRPDYWGQGTQVTVSSTTTPAPRPPTPAPTIASQPLSLRPEACRPAAGGAVHTRGLDFACDIYIWAPLAGTCGVLLLSLVITLYCKRGRKKLLYIFKQPFMRPVQTTQEEDGCSCRFPEEEEGGCELRVKFSRSADAPAYQQGQNQLYNELNLGRREEYDVLDKRRGRDPEMGGKPRRKNPQEGLYNELQKDKMAEAYSEIGMKGERRRGKGHDGLYQGLSTATKDTYDALHMQALPPR

SEQ ID NO: 36 - protein, 488 aa, synthetic construct
MALPVTALLLPLALLLHAARPDIQMTQTTSSLSASLGDRVTISCRASQDISKYLNWYQQKPDGTVKLLIYHTSRLHSGVPSRFSGSGSGTDYSLTISNLEQEDIATYFCQQGNTLPYTFGGGTKLEITGSTSGSGKPGSGEGSTKGEVKLQESGPGLVAPSQSLSVTCTVSGVSLPDYGVSWIRQPPRKGLEWLGVIWGSETTYYNSALKSRLTIIKDNSKSQVFLKMNSLQTDDTAIYYCAKHYYYGGSYAMDYWGQGTSVTVSSAAAIEVMYPPPYLDNEKSNGTIIHVKGKHLCPSPLFPGPSKPFWVLVVVGGVLACYSLLVTVAFIIFWVRSKRSRLLHSDYMNMTPRRPGPTRKHYQPYAPPRDFAAYRSRVKFSRSADAPAYQQGQNQLYNELNLGRREEYDVLDKRRGRDPEMGGKPRRKNPQEGLYNELQKDKMAEAYSEIGMKGERRRGKGHDGLYQGLSTATKDTYDALHMQALPPR

SEQ ID NO: 37 - protein, 491 aa, synthetic construct
MGQIVTFFQEVPHVIEEVMNIVLIALSVLAVLKGLYNFATCGLVGLVTFLLLCGRSCTTSLYKGVYELQTLELNMETLNMTMPLSCTKNNSHHYIMVGNETGLELTLTNTSIINHKFCNLSDAHKKNLYDHALMSIISTFALSIPNANQAEAMSCDFNGGKISVQYNLSHSYAGDAANHCGTVANGVLQTFMRMAWGGSYIALDSGRGNWDCIMTSYQYLIIQNTTWEDHCQFSRPSPIGYLGLLSQRTRDIYISRRLLGTFTWTLSDSEGKDTPGGYCLTRWMLIEAELKCFGNTAVAKCNEKHDEEFCDMLRLFDFNKQAIQRLKAEAQMSIQLINKAVNALINDQLIMKNHLRDIMGIPYCNYSKYWYLNHTTTGRTSLPKCWLVSNGSYLNETHFSDDIEQQADNMITEMLQKEYMERQGKTPLGLVDLFVFSTSFYLISIFLHLVKIPTHRHIVGKSCPKPHRLNHMGICSCGLYKQPGVPVKWKR

SEQ ID NO: 38 - protein, 511 aa, synthetic construct
MKCLLYLAFLFIGVNCKFTIVFPHNQKGNWKNVPSNYHYCPSSSDLNWHNDLIGTALQVKMPKSHKEIQADGWMCHASKWVTTCDFRWYGPKYITHSIRSFTPSVEQCKESIEQTKQGTWLNPGFPPQSCGYATVTDAEAVIVQVTPHHVLVDEYTGEWVDSQFINGKCSNYICPTVHNSTTWHSDYKVKGLCDSNLISMDITFFSEDGELSSLGKEGTGFRSNYFAYETGGKACKMQYCKHWGVRLPSGVWFEMADKDLFAAARFPECPEGSSISAPSQTSVDVSLIQDVERILDYSLCQETWSKIRAGLPISPVDLSYLAPKNPGTGPAFTIINGTLKYFETRYIRVDIAAPILSRMVGMISGTTTERELWDDWAPYEDVEIGPNGVLRTSSGYKFPLYMIGHGMLDSDLHLSSKAQVFEHPHIQDAASQLPDDESLFFGDTGLSKNPIELVEGWFSSWKSSIASFFFIIGLIIGLFLVLRVGIHLCIKLKHTKKRQIYTDIEMNRLGK

SEQ ID NO: 39 - protein, 511 aa, synthetic construct
MKCLLYLAFLFIGVNCKFTIVFPHNQKGNWKNVPSNYHYCPSSSDLNWHNDLIGTALQVKMPKSHKAIQADGWMCHASKWVTTCDFRWYGPKYITHSIRSFTPSVEQCKESIEQTKQGTWLNPGFPPQSCGYATVTDAEAVIVQVTPHHVLVDEYTGEWVDSQFINGKCSNYICPTVHNSTTWHSDYKVKGLCDSNLESMDITFFSEDGELSSLGKEGTGFRSNYFAYETGGKACKMQYCKHWGVRLPSGVWFEMADKDLFAAARFPECPEGSSISAPSQTSVDVSLIQDVERILDYSLCQETWSKIRAGLPISPVDLSYLAPKNPGTGPAFTIINGTLKYFETRYIRVDIAAPILSRMVGMISGTTTERELWDDWAPYEDVEIGPNGVLRTSSGYKFPLYMIGHGMLDSDLHLSSKAQVFEHPHIQDAASQLPDDESLFFGDTGLSKNPIELVEGWFSSWKSSIASFFFIIGLIIGLFLVLRVGIHLCIKLKHTKKRQIYTDIEMNRLGK

SEQ ID NO: 40 - protein, 511 aa, synthetic construct
MKCLLYLAFLFIGVNCKFTIVFPHNQKGNWKNVPSNYHYCPSSSDLNWHNDLIGTALQVKMPKSHKAIQADGWMCHASKWVTTCDFRWYGPKYITHSIRSFTPSVEQCKESIEQTKQGTWLNPGFPPQSCGYATVTDAEAVIVQVTPHHVLVDEYTGEWVDSQFINGKCSNYICPTVHNSTTWHSDYKVKGLCDSNLISMDITFFSEDGELSSLGKEGTGFRSNYFAYETGGKACKMQYCKHWGVRLPSGVWFEMADKDLFAAARFPECPEGSSISAPSQTSVDVSLIQDVERILDYSLCQETWSKIRAGLPISPVDLSYLAPKNPGTGPAFTIINGTLKYFETRYERVDIAAPILSRMVGMISGTTTERELWDDWAPYEDVEIGPNGVLRTSSGYKFPLYMIGHGMLDSDLHLSSKAQVFEHPHIQDAASQLPDDESLFFGDTGLSKNPIELVEGWFSSWKSSIASFFFIIGLIIGLFLVLRVGIHLCIKLKHTKKRQIYTDIEMNRLGK

SEQ ID NO: 41 - protein, 262 aa, synthetic construct
METDTLLLWVLLLWVPGSTGDDVQLQQSGPGLVKPSQSLSLTCTVTGYSITSDSAWNWIRQFPGNRLEWMGYISYSGSTSYNPSLKSRISITRDTSKNQFFLQLNSVTTEDTATYYCVRGLRFAYWGQGTLVTVSSGGGGSGGGGSGGGGSDIVLTQSPASLAVSLGQRATISCRASESVDSYVNSFLHWYQQKPGQPPKLLIYRASNLQSGIPARFSGSGSRTDFTLTINPVEADDVATYYCQQSNEDPYTFGGGTKLEIK

SEQ ID NO: 42 - protein, 52 aa, synthetic construct
LQSRPEPTAPPEEDPAVDLLKNYPSQKQEPIDKELYPLASLRSLFGSDPSSQ

SEQ ID NO: 43 - protein, 112 aa, synthetic construct
MSDPRERIPPGNSGEETIGEAFEWLNRTVEEINREAVNHLPRELIFQVWQRSWEYWHDEQGMSPSYVKYRYLCLIQKALFMHCKKGCRCLGEGHGAGGWRPGPPPPPPPGLA

SEQ ID NO: 44 - protein, 187 aa, synthetic construct
METDTLLLWVLLLWVPGSTGDEVQLVESGGGLVQPGGSLRLSCAASGDVHKINILGWYRQAPAKEREMVAHITIGDATDYADSAKGRFTISRDEAKNMVYLQMNSLKPEDTAVYFCRAYSRIYPYNYWGQGTLVTVSSAVGQDTQEVIVVPHSLPFKVVVISAILALVVLTIISLIILIMLWQKKPR

SEQ ID NO: 45 - protein, 218 aa, synthetic construct
METDTLLLWVLLLWVPGSTGDEVQLVESGGGLVQPGGSLRLSCAASGDVHKINILGWYRQAPAKEREMVAHITIGDATDYADSAKGRFTISRDEAKNMVYLQMNSLKPEDTAVYFCRAYSRIYPYNYWGQGTLVTVSSPAKPTTTPAPRPPTPAPTIASQPLSLRPEACRPAAGGAVHTRGLDFACDIVVVISAILALVVLTIISLIILIMLWQKKPR

SEQ ID NO: 46 - protein, 207 aa, synthetic construct
METDTLLLWVLLLWVPGSTGDEVQLVESGGGLVQPGGSLRLSCAASGDVHKINILGWYRQAPAKEREMVAHITIGDATDYADSAKGRFTISRDEAKNMVYLQMNSLKPEDTAVYFCRAYSRIYPYNYWGQGTLVTVSSASGGGGSGELAAIKQELAAIKKELAAIKWELAAIKQGAGVVVISAILALVVLTIISLIILIMLWQKKPR

SEQ ID NO: 47 - protein, 511 aa, synthetic construct
MKCLLYLAFLFIGVNCKFTIVFPHNQKGNWKNVPSNYHYCPSSSDLNWHNDLIGTALQVKMPASHKAIQADGWMCHASKWVTTCDFRWYGPKYITHSIRSFTPSVEQCKESIEQTKQGTWLNPGFPPQSCGYATVTDAEAVIVQVTPHHVLVDEYTGEWVDSQFINGKCSNYICPTVHNSTTWHSDYKVKGLCDSNLISMDITFFSEDGELSSLGKEGTGFRSNYFAYETGGKACKMQYCKHWGVRLPSGVWFEMADKDLFAAARFPECPEGSSISAPSQTSVDVSLIQDVERILDYSLCQETWSKIRAGLPISPVDLSYLAPKNPGTGPAFTIINGTLKYFETRYIRVDIAAPILSRMVGMISGTTTEAELWDDWAPYEDVEIGPNGVLRTSSGYKFPLYMIGHGMLDSDLHLSSKAQVFEHPHIQDAASQLPDDESLFFGDTGLSKNPIELVEGWFSSWKSSIASFFFIIGLIIGLFLVLRVGIHLCIKLKHTKKRQIYTDIEMNRLGK

SEQ ID NO: 48 - protein, 323 aa, synthetic construct
MEWSWIFLFLLSGTAGVHSGKPIPNPLLGLDSTEVQLQQSGPELVKPGASVKMSCKASGYKFTSYVMHWVKQKPGQGLEWIGYINPYNDVTKYNEKFKGKATLTSDKSSSTAYMELSSLTSEDSAVHYCARGSYYDYDGFVYWGQGTLVTVSAGGGGSGGGGSGGGGSQIVLTQSPAIMSASPGEKVTMTCSATSSVSYMHWYQQKSGTSPKRWIYDTSKLASGVPARFSGSGSGTSYSLTISSMEAEDAATYYCQQWSSNPLTFGAGTKLELKAVGQDTQEVIVVPHSLPFKVVVISAILALVVLTIISLIILIMLWQKKPR

SEQ ID NO: 49 - protein, 337 aa, synthetic construct
MEWSWIFLFLLSGTAGVHSGKPIPNPLLGLDSTEVQLQQSGPELVKPGASVKMSCKASGYKFTSYVMHWVKQKPGQGLEWIGYINPYNDVTKYNEKFKGKATLTSDKSSSTAYMELSSLTSEDSAVHYCARGSYYDYDGFVYWGQGTLVTVSAGGGGSGGGGSGGGGSQIVLTQSPAIMSASPGEKVTMTCSATSSVSYMHWYQQKSGTSPKRWIYDTSKLASGVPARFSGSGSGTSYSLTISSMEAEDAATYYCQQWSSNPLTFGAGTKLELKASESKYGPPCPPCPAVGQDTQEVIVVPHSLPFKVVVISAILALVVLTIISLIILIMLWQKKPR

SEQ ID NO: 50 - protein, 177 aa, synthetic construct
METDTLLLWVLLLWVPGSTGDAAPLKIQAYFNETADLPCQFANSQNQSLSELVVFWQDQENLVLNEVYLGKEKFDSVHSKYMGRTSFDSDSWTLRLHNLQIKDKGLYQCIIHHKKPTGMIRIHQMNSELSVLSASESKYGPPCPPCPVVVISAILALVVLTIISLIILIMLWQKKPR

SEQ ID NO: 51 - protein, 308 aa, synthetic construct
METDTLLLWVLLLWVPGSTGDQVQLVQSGAEVKKPGASVKVSCKASGYTFTSYYIHWVRQAPGQGLEWIGCIYPGNVNTNYNEKFKDRATLTVDTSISTAYMELSRLRSDDTAVYFCTRSHYGLDWNFDVWGQGTTVTVSSGGGGSGGGGSGGGGSDIQMTQSPSSLSASVGDRVTITCHASQNIYVWLNWYQQKPGKAPKLLIYKASNLHTGVPSRFSGSGSGTDFTLTISSLQPEDFATYYCQQGQTYPYTFGGGTKVEIKSASESKYGPPCPPCPVVVISAILALVVLTIISLIILIMLWQKKPR

SEQ ID NO: 52 - protein, 218 aa, synthetic construct
METDTLLLWVLLLWVPGSTGDEVQLVESGGGLVQPGGSLRLSCAASGDVHKINILGWYRQAPAKEREMVAHITIGDATDYADSAKGRFTISRDEAKNMVYLQMNSLKPEDTAVYFCRAYSRIYPYNYWGQGTLVTVSSGASAKPTTTPAPRPPTPAPTIASQPLSLRPEAARPAAGGAVHTRGLDFAKVVVISAILALVVLTIISLIILIMLWQKKPR

SEQ ID NO: 53 - protein, 494 aa, synthetic construct
MALPVTALLLPLALLLHAARPQVQLQESGPGLIKPSQTLSLTCTVSGGSISSGYNWHWIRQPPGKGLEWIGYIHYTGSTNYNPALRSRVTISVDTSKNQFSLKLSSVTAADTAIYYCARIYNGNSFPYWGQGTTVTVSSGGGGSGGGGSGGGGSDIVMTQSPDSLAVSLGERATINCKSSQSLFNSGNQKNYLTWYQQKPGQPPKLLIYWASTRESGVPDRFSGSGSGTDFTLTISSLQAEDVAVYYCQNAYSFPYTFGGGTKLEIKRTTTPAPRPPTPAPTIASQPLSLRPEACRPAAGGAVHTRGLDFACDFWVLVVVGGVLACYSLLVTVAFIIFWVRSKRSRLLHSDYMNMTPRRPGPTRKHYQPYAPPRDFAAYRSRVKFSRSADAPAYQQGQNQLYNELNLGRREEYDVLDKRRGRDPEMGGKPQRRKNPQEGLYNELQKDKMAEAYSEIGMKGERRRGKGHDGLYQGLSTATKDTYDALHMQALPPR

SEQ ID NO: 54 - protein, 117 aa, synthetic construct
EVQLVESGGGLVQPGGSLRLSCAASGDVHHINILGWYRQAPAKEREMVAHITIGDATDYADSAKGRFTISRDEAKNMVYLQMNSLKPEDTAVYFCRADSRIYPYNYWGQGTLVTVSS

SEQ ID NO: 55 - protein, 117 aa, synthetic construct
EVQLVESGGGLVQPGGSLRLSCAASGDVSKINILGWYRQAPAKEREMVAHITIGDITDYADSAKGRFTISRDEAKNMVYLQMNSLKPEDTAVYFCRALSRIYPYNYWGQGTLVTVSS

SEQ ID NO: 56 - protein, 117 aa, synthetic construct
EVQLVESGGGLVQPGGSLRLSCAASGDVLKINILGWYRQAPAKEREMVAHITIGDAEDYADSAKGRFTISRDEAKNMVYLQMNSLKPEDTAVYFCRALSRIYPYNYWGQGTLVTVSS

SEQ ID NO: 57 - protein, 117 aa, synthetic construct
EVQLVESGGGLVQPGGSLRLSCAASGDVHKINILGWYRQAPAKEREMVAHITSGDATDYADSAKGRFTISRDEAKNMVYLQMNSLKPEDTAVYFCRAYSRIYPYNYWGQGTLVTVSS

SEQ ID NO: 58 - protein, 117 aa, synthetic construct
EVQLVESGGGLVQPGGSLRLSCAASGDVHVINILGWYRQAPAKEREMVAHITIGDKTDYADSAKGRFTISRDEAKNMVYLQMNSLKPEDTAVYFCRAYSRIYPYNYWGQGTLVTVSS

SEQ ID NO: 59 - protein, 117 aa, synthetic construct
EVQLVESGGGLVQPGGSLRLSCAASGDVHKINILGWYRQAPAKEREMVAHITYGDATDYADSAKGRFTISRDEAKNMVYLQMNSLKPEDTAVYFCVAYSRIYPYNYWGQGTLVTVSS

SEQ ID NO: 60 - protein, 117 aa, synthetic construct
EVQLVESGGGLVQPGGSLRLSCAASGDVRKINILGWYRQAPAKEREMVAHIHIGDATDYADSAKGRFTISRDEAKNMVYLQMNSLKPEDTAVYFCTAYSRIYPYNYWGQGTLVTVSS

SEQ ID NO: 61 - protein, 117 aa, synthetic construct
EVQLVESGGGLVQPGGSLRLSCAASLDVHKINILGWYRQAPAKEREMVAHITIGDATDYADSAKGRFTISRDEAKNMVYLQMNSLKPEDTAVYFCRAYSRIYPYNYWGQGTLVTVSS

SEQ ID NO: 62 - protein, 117 aa, synthetic construct
EVQLVESGGGLVQPGGSLRLSCAASGDVHRINILGWYRQAPAKEREMVAHITIGDATDYADSAKGRFTISRDEAKNMVYLQMNSLKPEDTAVYFCRAYSRIYPYNYWGQGTLVTVSS

SEQ ID NO: 63 - protein, 117 aa, synthetic construct
EVQLVESGGGLVQPGGSLRLSCAASGDVPKINILGWYRQAPAKEREMVAHITIGDATDYADSAKGRFTISRDEAKNMVYLQMNSLKPEDTAVYFCRAYSRIYPYNYWGQGTLVTVSS

SEQ ID NO: 64 - protein, 117 aa, synthetic construct
EVQLVESGGGLVQPGGSLRLSCAASGDVHVINILGWYRQAPAKEREMVAHITIGEATDYADSAKGRFTISRDEAKNMVYLQMNSLKPEDTAVYFCSAYSRIYPYNYWGQGTLVTVSS

SEQ ID NO: 65 - protein, 117 aa, synthetic construct
EVQLVESGGGLVQPGGSLRLSCAASGDVHTINILGWYRQAPAKEREMVAHITIGDAPDYADSAKGRFTISRDEAKNMVYLQMNSLKPEDTAVYFCRAYSRLYPYNYWGQGTLVTVSS

SEQ ID NO: 66 - protein, 115 aa, synthetic construct
QVQLQESGGGLVQPGGSLRLSCAASGFTFSSYAMSWVRQAPGKGLEWVSVINSGGGRTKYADSVKGRFTISRDNAKNTLYLQMNSLRPEDTAVYYCALGRDWSQRGQGTQVTVSS

SEQ ID NO: 67 - protein, 115 aa, synthetic construct
QVQLQESGGGLVQPGGSLRLSCAASGFTFSSYAMSWVRQAPGKGLEWVSVINSGGGSTRYADSVKGRFTISRDNAKNTLYLQMNSLRPEDTAVYYCALGRDWSQRGQGTQVIVSS

SEQ ID NO: 68 - protein, 115 aa, synthetic construct
QVQLQESGGGLVQPGGSLRLSCAASGFTFSSYAMSWVRQAPGKGLEWVSVINTGGGRTRYADSVKGRFTISRDNAKNTLYLQMNSLRPEDTAVYYCALGRDWSQRGQGTQVTVSS

SEQ ID NO: 69 - protein, 115 aa, synthetic construct
QVQLQESGGGLVQPGGSLRLSCAASGFTFSMYAMTWVRQAPGKGLEWVSAITSGGGTTRYADSVKGRFTISRDNAKNTLYLQMNSLKADDTAVYYCALGRDWSQRGQGTQVTVSS

SEQ ID NO: 70 - protein, 115 aa, synthetic construct
QVQLQESGGGLVQAGGSLRLSCAASGRIFSIRPMGWYRQAPGKEREMVAQISSSGITNYGDSVKGRFTISRGNARNTVYLQMNNLKPEDTAVYYCRLFKTGADSWGQGTQVTVSS

SEQ ID NO: 71 - protein, 115 aa, synthetic construct
QVQLQESGGGLVQAGGSLRLSCAASGRIFSIRPMGWYRQPPGKEREMVAQISSNGITNYGDSVKGRFTISRGSARNTVYLQMNNLKPEDTAVYYCRLFKTGADSWGQGTQVTVSS

SEQ ID NO: 72 - protein, 115 aa, synthetic construct
QVQLQESGGGLVQAGGSLRLSCAASGRIFSIRPMGWYRQPPGKEREMVAQISSSGITNYGDSVKGRFTISRGNARNTVYLQMNNLKPEDTAVYYCRLFKTGADSWGQGTQVTVSS

SEQ ID NO: 73 - protein, 122 aa, synthetic construct
QVQLQESGGGLVQAGGSLRLSCVASGNIRSVGDMGWYRQTLGDQREMVATIDYGGVARYADAVKGRFTISRDNAKSAVYLQMNSLNREDTAVYYCNADILYKSDSYARREFWGQGTQVTVSS

SEQ ID NO: 74 - protein, 122 aa, synthetic construct
QVQLQESGGGLVQPGGSLRLSCVASGNIRSVGDMGWYRQTLGDQREMVATIDYGGVARYADAVKGRFTISRDNAKSAVYLQMNSLNREDTAVYYCNADILYKSDSYARREFWGQGTQVTVSS

SEQ ID NO: 75 - protein, 122 aa, synthetic construct
QVQLQESGGGSVQTGESLRLSCVASGNIRSVGDMGWYRQTLGDQREMVATIDYGGVARYADAVKGRFTISRDNAKSAVYLQMNSLNREDTAVYYCNADILYKSDSYARREFWGQGTQVTVSS

SEQ ID NO: 76 - protein, 122 aa, synthetic construct
QVQLQESGGGLVQSGGSLRLSCAVSGSIFSIVDMGWYRQAPGKGRELVAELSDGSTNYADSVLGRFTISRDNAKNTVYLQMNSLKPEDTAVYYCNADLTGSSWSPYRYLEVWGQGTQVTVSS

SEQ ID NO: 77 - protein, 122 aa, synthetic construct
QVQLQESGGGLVQSGGSLRLSCAVSVSIFSIVDMGWYRQAPGKGRELVAELSGGSTNYADSVLGRFTISRDNAKNTVYLQMNSLKPEDTAVYYCNADLTGSSWYPYRFLEVWGQGTQVTVSS

SEQ ID NO: 78 - protein, 122 aa, synthetic construct
QVQLQESGGGLVQSGGSLRLSCAVSSSIFSIVDMGWYRQAPGKGRELVAELSVGSTNYADSVLGRFTISRDNAKNTVYLQMNSLKPEDTAVYYCNADLTGSSLSPYRYLEVWGQGTQVTVSS

SEQ ID NO: 79 - protein, 122 aa, synthetic construct
QVQLQESGGGLVQSGGSLRLSCAVSGSIFSIVDMGWYRQAPGKGRELVAELSDGSSNYADSVLGRFTISRDNAKNTVYLQMNSLKPEDTAVYYCYADLTGSSWSPYRYLEVWGQGTQVTVSS

SEQ ID NO: 80 - protein, 122 aa, synthetic construct
QVQLQESGGGLVQSGGSLRLSCAVSGSIFSIVDMGWYRQAPGKGRELVAELSSGSTNYADSVLGRFTISRDNAKNTVYLQMNSLKPEDTAVYYCNEDLTGSSWSPYRYLEVWGQGTQVTVSS

SEQ ID NO: 81 - protein, 122 aa, synthetic construct
QVQLQESGGGLVQSGGSLRLSCAVSGSIFSILDMGWYRQAPGKGRELVAELSNGSTNYADSVLGRFTISRDNAKNTVYLQMNSLKPEDTAVYYCNADLTGSSVSPYRYLEVWGQGTQVTDSS

SEQ ID NO: 82 - protein, 122 aa, synthetic construct
QVQLQESGGGLVQSGGSLRLSCAVSRSIFSIVDMGWYRQAPGKGRELVAELSDGSRNYADSVLGRFTISRDNAKNTVYLQMNSLKPEDTAVYYCNDDLTGSSWSPYRYLEVWGQGTQVTVSS

SEQ ID NO: 83 - protein, 122 aa, synthetic construct
QVQLQESGGGLVQSGGSLRLSCAVSGSSFSIVDMGWYRQAPGKGRELVAELSDGSTNYADSVLGRFTISRDNAKNTVYLQMNSLKPEDTAVYYCNADLTGSSFSPYRYLEVWGQGTQVTVSS

SEQ ID NO: 84 - protein, 122 aa, synthetic construct
QVQLQESGGGLVQSGGSLRLSCAVSGSIFSIVDMGWYRQAPGKGRELVAELSDGSSNYADSVLGRFTISRDNAKNTVYLQMNSLKPEDTAVYYCNADLTGSSWSRYRYLEVWGQGTQVTVSS

SEQ ID NO: 85 - protein, 122 aa, synthetic construct
QVQLQDSGGGLVQSGGSLRLSCAVSGSIFSIVDMGWYRQAPGKGRELVAELSVGSTNYADSVLGRFTISRDNAKNTVYLQMNSLKPEDTAVYYCNADLTGSSWSPYRYQEVWGQGTQVTVSS

SEQ ID NO: 86 - protein, 122 aa, synthetic construct
QVQLQESGGGLVQSGGSLRLSCAVSGSIFSIVDMGWYRQAPGKGRELVAELSYGSTNYADSVLGRFTISRDNAKNTVYLQMNSLKPEDTAVYYCNADLTGTSWSPYRYLEVWGQGTQVTVSS

SEQ ID NO: 87 - protein, 122 aa, synthetic construct
QVQLQESGGGLVQSGGSLRLSCAVSGSIFSIVEMGWYRQAPGKGRELVAELSDGVTNYADSVLGRFTISRDNAKNTVYLQMNSLKPEDTAVYYCTADLTGSSWSPYRYLEVWGQGTQVTVSS

SEQ ID NO: 88 - protein, 122 aa, synthetic construct
QVQLQESGGGLVQSGGSLRLSCAVSGSIFSIVDMGWYRQAPGKGRELVAELSDGSCNYADSVLGRFTISRDNAKNTVYLQMNSLKPEDTAVYYCNADLTGSLWSPYRYLEVWGQGTQVTVSS

SEQ ID NO: 89 - protein, 122 aa, synthetic construct
QVQLQESGGGLVQSGGSLRLSCAVSGSIFSMVDMGWYRQAPGKGRELVAELSLGSTNYADSVLGRFTISRDNAKNTVYLQMNSLKPEDTAVYYCNADLTGSSWEPYRYLEVWGQGTQVTVSS

SEQ ID NO: 90 - protein, 122 aa, synthetic construct
QVQLQESGGGLVQSGGSLRLSCAVSGSIFSILDMGWYRQAPGKGRELVAELSDGSTNYADSVLGRFTISRDNAKNTVYLQMNSLKPEDTAVYYCNADLTGSSWSEYRYLEVWGQGTQVTVSS

SEQ ID NO: 91 - protein, 122 aa, synthetic construct
QVQLQESGGGLVQSGGSLRLSCAVSGSLFSIVDMGWYRQAPGKGRELVAELSDGPTNYADSVLGRFTISRDNAKNTVYLQMNSLKPEDTAVYYCNADLTGSSWSLYRYLEHWGQGTQVTVSS

SEQ ID NO: 92 - protein, 122 aa, synthetic construct
QVQLQESGGGLVQSGGSLRLSCAVSGSIFSIVDMGWYRQAPGKGRELVAELSDGCTNYADSVLGRFTISRDNAKNTVYLQMNSLKPEDTAVYYCNIDLTGSSWSPYRYLEVWGQGTQVTVSS

SEQ ID NO: 93 - protein, 122 aa, synthetic construct
QVQLQESGGGLVQSGGSLRLSCAVSGSIFSIVDMGWYRQAPGKGRELVAELSSGSTNYADSVLGRFTISRDNAKNTVYLQMNSLKPEDTAVYYCNADLTGSSWSPYRYLEVWGQGTQVTVSS

SEQ ID NO: 94 - protein, 122 aa, synthetic construct
QVQLQESGGGLVQSGGSLRLSCAVSGSIFSIVDMGWYRQAPGKGRELVAELSGGSTNYADSVLGRFTISRDNAKNTVYLQMNSLKPEDTAVYYCNADLTGSSWSPYRYLEVWGQGTQVTVSS

SEQ ID NO: 95 - protein, 122 aa, synthetic construct
QVQLQESGGGLVQSGGSLRLSCAVSGSIFSIVDMGWYRQAPGKGRELVAELSDGATNYADSVLGRFTISRDNAKNTVYLQMNSLKPEDTAVYYCNADLTGSSYSPYRYLEVWGQGTQVTVSS

SEQ ID NO: 96 - protein, 122 aa, synthetic construct
QVQLQESGGGLVQSGGSLRLSCAVSGSIFSIVDMGWYRQAPGKGRELVAELSDSSTNYADSVLGRFTISRDNAKNTVYLQMNSLKPEDTAVYYCNADLTGSSWSPYRYLEVWGQGTQVTVSS

SEQ ID NO: 97 - protein, 122 aa, synthetic construct
QVQLQESGGGLVQSGGSLRLSCSVSGSFFSIVDMGWYRQAPGKGRELVAELSDGSTNYADSVLGRFTISRDNAKNTVYLQMNSLKPEDTAVYYCNADLTGSSWSPYRYLEVWGQGTQVTVSS

SEQ ID NO: 98 - protein, 122 aa, synthetic construct
QVQLQESGGGLVQSGGSLRLSCAVSGSIFSIVDMGWYRQAPGKGRELVAELYDGSTNYADSVLGRFTISRDNAKNTVYLQMNSLKPEDTAVYYCNADLTGSYWSPYRYLEVWGQGTQVTVSS

SEQ ID NO: 99 - protein, 122 aa, synthetic construct
QVQLQESGGGLVQSGGSLRLSCAVSGSSFSIVDMGWYRQAPGKGRELVAEISDGSTNYADSVLGRFTISRDNAKNTVYLQMNSLKPEDTAVYYCNADLTGSSWSPYRYLEVWGQGTQVTVSS

SEQ ID NO: 100 - protein, 122 aa, synthetic construct
QVQLQESGGGLVQSGGSLRLSCAVSGSIFSIVDMGWYRQAPGKGRELVAELSDASTNYADSVLGRFTISRDNAKNTVYLQMNSLKPEDTAVYYCYADLTGSSWSPYRYLEVWGQGTQVTVSS

SEQ ID NO: 101 - protein, 122 aa, synthetic construct
QVQLQESGGGLVQSGGSLRLSCAVSGSLFSIVDMGWYRQAPGKGRELVAELSDGLTNYADSVLGRFTISRDNAKNTVYLQMNSLKPEDTAVYYCNADLTGSSWSPYRYLEVWGQGTQVTVSS

SEQ ID NO: 102 - protein, 123 aa, synthetic construct
QVQLQESGGGLVQPGGSLRLSCAASGSIFSTNAMSWYRQAPGKERELVAEITSGGSTNYADSVKGRFTISRDNAKNTVYLQMNSLKPEDTAVYYCNADLTGSSWSPYRYLEVWGQGTQVTVSS

SEQ ID NO: 103 - protein, 124 aa, synthetic construct
QVQLQESGGGLVQPGGSLRLSCSASESVKSINVMGWYRQAPGKERESVAAISAEGRTNYTDSVKGRFTISRDKGKDTVYLQMNDLKPEDTAVYYCHADRILYKTDLYYVKNDVWGQGTQVTVSS

SEQ ID NO: 104 - protein, 124 aa, synthetic construct
QVQLQESGGGLVQLGGSLRLSCSASESVKSINVMGWYRQAPGKERESVAAISAEGRTNYTDSVKGRFTISRDKGKDTVYLQMNDLKPEDTAVYYCHADRILYKTDLYYVKNDVWGQGTQVTVSS

SEQ ID NO: 105 - protein, 116 aa, synthetic construct
QVQLQESGGGLVQAGESLTLSCQPSERISRIDVLGWYRQAPDKDRELVALSGKGGRTYYADSVKDRFTISRDTANNRLYLQMNKLEVDDTAIYYCVTEAEGGGYTSGQGTQVTVSS

SEQ ID NO: 106 - protein, 119 aa, synthetic construct
QVQLQESGGGLVQAGDSLTISCAASGAASTFTLMAWYRQAPGKQRKLVGSITGSGRTAYAQSLKDRFTISRTDAKDTMYLQMNNLKPEDTAVYYCNAISTNGGTMEDYWGQGTQVTVSS

SEQ ID NO: 107 - protein, 122 aa, synthetic construct
QVQLQESGGGLVQSGGSLRLSCTVTGRIPARYSLGWYRQLPGKEREFVAAINWNGDNTYYENSVKGRFTISRDNTKNTVDLQMRSLRVEDTAVYYCAASGHSDYIDNGFGTFGQGTQVTVSS

SEQ ID NO: 108 - protein, 125 aa, synthetic construct
QVQLQESGGGLVQPGGSLRLSCAASGRTFSIYAMGWFRQAPGKEHDFVAAISWSGGNTYYADSVKGRFTISRDNAKNTVYLQMNSLKPEDTAVYYCAATTHIPYSDYDADEYDYWGQGTQVTVSS

SEQ ID NO: 109 - protein, 126 aa, synthetic construct
QVQLQESGGGSVQAGGSLRLSCTTSRPISSIYAMGWFRQAPGTERESVAAINWSSGNGYYADSVKGRFTISRDNAKKTVYLQMNNLKSEDTAVYYCAAARQATGWSILTAAAHEYWGQGTQVTVSS

SEQ ID NO: 110 - protein, 127 aa, synthetic construct
QVQLQESGGGLVQAGGSLRLSCAASGRTFSSYAMGWFRQAPGKERAFVAAISWSGGNTDYADSVKGRFTISRDNAKNTVYLQMNSLKPEDTAVYYCAADRRDLYGSRWYAAGWYDYWGQGTQVTVSS

SEQ ID NO: 111 - protein, 130 aa, synthetic construct
QVQLQESGGGLVAPGGSLRLSCVAAGSRFGFDYYAIGWFRQALGRQREMVSCISGSGRGSNYADSVKGRFTISRDNAKNTVYLQMESLKPEDTDVYYCGAVYSPVYSDLALCRLDSISTWGQGTQVTVSS

SEQ ID NO: 112 - protein, 129 aa, synthetic construct
QVQLQESGGGLVQSGDSLKLSCHDPGAIIVGQTVAWFRQVPGKEREGIACITWDSNWKNYADSVKDRFTISRDNSKKEIYLQMDSLKPEDTAVYYCAGDEYLNYCDSPRAFQRGTYDYWGQGTQVTVSS

SEQ ID NO: 113 - protein, 112 aa, synthetic construct
QVQLQESGGGLVQTGGSLRLSCTASGQTFSDNTMAWWRQAPGKQREMVAIITRNNKTTYGDSVKGRFTISRDIPKNMVFLQMNNLNSEDTGVYYCNAGFVYWGQGTQVTVSS

SEQ ID NO: 114 - protein, 114 aa, synthetic construct
QVQLQESGGGSVQAGGSLRLSCVASGASSFIALGWYRQVPGKLRELVARIVDTGSINYADHVKGRFTISRDNAKNALYLEMNSLKPEDTAIYYCKMNTKYDVYWGQGTQVTVSS

SEQ ID NO: 115 - protein, 118 aa, synthetic construct
QVQLQESGGGSVQPGGSLRLSCSRSGPIYSVDTMGWYRRAPGEQRELVASITVGGTTTYADSVKGRFTISRDNTMNTVYLQMNNLKIEDTDVYYCNLNRRLAKSEDYWGRGTQVTVSS

SEQ ID NO: 116 - protein, 119 aa, synthetic construct
QVQLQESGGGLVQAGGSLRLSCTVSGASFTFNAMGWYRQAPGKQRELVARITKSGTIDYADSVKGRFTISGDSHNNAVYLKMNTLELDDTGVYYCYARLYYMHSWFDVYGKGTQVTVSS

SEQ ID NO: 117 - protein, 125 aa, synthetic construct
QVQLQESGGGLVQSGESLRLSCTTSGDIFGVTGVGWYRQAPGKQRELVAALSNEGYTNYKDPVKGRFTISRDNNKTAVYLQMNDLKPEDTAVYYCKVHCTSSGCQFVGHQSFDYWGQGTQVTVSS

SEQ ID NO: 118 - protein, 124 aa, synthetic construct
QVQLQESGGGLVQTGGSLRLSCAASGRTFSNYAMGWFRQAPGKGRAFIGGISRSGGNTHFADSVMGRFTISRDNAKNTVYLQMNSLTPEDTAVYYCAAQYQWTEAVPLGNYNIWGQGTQVTVSS

SEQ ID NO: 119 - protein, 122 aa, synthetic construct
QVQLQESGGGLVQPGGSLRLSCAASGSSTSINAMGWYRQAPGKERELVARITGSGSTSYSDSVKGRFTISRDNAKNTVYLQMNSLKAEDTAVYYCGASRFRVGSQRTEYGYWGQGTQVTVSS

SEQ ID NO: 120 - protein, 115 aa, synthetic construct
QVQLQESGGGLAQPGGSLRLSCTSSISIFRLNSMGWYRQTPGKERELVATITNGGTVNYADSVKGRFTISRDNAKNTVYLQMNSLKSEDTAVYYCKSWPFPQEYWGKGTQVTVSS

SEQ ID NO: 121 - protein, 119 aa, synthetic construct
QVQLQESGGGSVQPGGSLRLSCVVSGFTTDNYIIAWYRQAPGKGREGVSSISRSDGSTYYAPSVKGRFSITSDSAKNTVSLQMNSLKPEDTAVYYCNAHDSYGNERDYWGQGTQVTVSS

SEQ ID NO: 122 - DNA, 910 bp, synthetic construct
  source 1..910: mol_type = other DNA
gggaagatgtgagacaaacatcacaattttgcctaaggtgaatccaacccacaagtagagcacaggccaacagcagctcactagtacacatacttacaccagcagctcactagtacacacacttacaccagacgctcactggtacacactcacaccggcattcatgcttacccacgggctggtcaacaaagaggtgctgacctgagagtagggcacataacctcagccactggggtacacttaccacccccgcccccgtgtagctccctcccctatcctgaaatctcccttagcacactaagtattctaggttaaacagcccagatgttcagggagttcattcgccaggtgggaagtaatgagatgtaaatcggggtcttttaggtaatagctgacaactggggtaggaatgggggttctgagcccagtgctggctgccgggctgtttatctctgagtcacatcagcaccaagccacagcagccacctgccctagctccatctcttacagtcacaacaggatgtggtttgacatttactgggtcctgcatctggggtgcctgtgaaagttgctccctccacccacccaccttcagagcatcatgagaaccacactcaccgcatccggcacccaaccccctcctatgctgctctttctacctgggcccctggttagcatcctggcagtagaaatagaatttacaccgcttccttcctaccctacccctagcccacccccactctgaaaatttcccaccatcaacggcagaaagcagagaagcagacatcttctagttcctcccccactctcctctttccggtacctgtgagtcagctaggggagggcagctctcacccaggctgatagttcggtgacctggctttatctactggatgagttccgctgggag

SEQ ID NO: 123 - DNA, 719 bp, synthetic construct
  source 1..719: mol_type = other DNA
gggaagatgtgagacaaacatcacaattttgcctaaggtgaatccaacccacaagtagagcacaggccaacagcagctcactagtacacatacttacaccagcagctcactagtacacacacttacaccagacgctcactggtacacactcacaccggtgggaagtaatgagatgtaaatcggggtcttttaggtaatagctgacaactggggtaggaatgggggttctgagcccagtgctggctgccgggctgtttatctctgagtcacatcagcaccaagccacagcagccacctgccctagctccatctcttacagtcacaacaggatgtggtttgacatttactgggtcctgcatctggggtgcctgtgaaagttgctccctccacccacccaccttcagagcatcatgagaaccacactcaccgcatccggcacccaaccccctcctatgctgctctttctacctgggcccctggttagcatcctggcagtagaaatagaatttacaccgcttccttcctaccctacccctagcccacccccactctgaaaatttcccaccatcaacggcagaaagcagagaagcagacatcttctagttcctcccccactctcctctttccggtacctgtgagtcagctaggggagggcagctctcacccaggctgatagttcggtgacctggctttatctactggatgagttccgctgggag

SEQ ID NO: 124 - DNA, 719 bp, synthetic construct
  source 1..719: mol_type = other DNA
ggtgggaagtaatgagatgtaaatcggggtcttttaggtaatagctgacaactggggtaggaatgggggttctgagcccagtgctggctgccgggctgtttatctctgagtcacatcagcaccaagccacagcagccacctgccctagctccatctcttacagtcacaacaggatgtggtttgacatttactgggtcctgcatctggggtgcctgtgaaagttgctccctccacccacccaccttcagagcatcatgagaaccacactcaccgcatccggcacccaaccccctcctatgctgctctttctacctgggcccctggttagcatcctggcagtagaaatagaagggaagatgtgagacaaacatcacaattttgcctaaggtgaatccaacccacaagtagagcacaggccaacagcagctcactagtacacatacttacaccagcagctcactagtacacacacttacaccagacgctcactggtacacactcacacctttacaccgcttccttcctaccctacccctagcccacccccactctgaaaatttcccaccatcaacggcagaaagcagagaagcagacatcttctagttcctcccccactctcctctttccggtacctgtgagtcagctaggggagggcagctctcacccaggctgatagttcggtgacctggctttatctactggatgagttccgctgggag

SEQ ID NO: 125 - DNA, 945 bp, synthetic construct
  source 1..945: mol_type = other DNA
aaataaacaaggagatagggtgtttattttatggacaagtttcttttgtaacttgtaactcccttgaaagtcagccagagtatgtctcaaaccaaagtcaagatagtgagcaagaagtgttgcacttatgaagggaggtgagtgagcaatgcatgtggtttccaaccgttaatgctagagttatcactttctgttatcaagtggcttcagctatgcaaggaaaccaaacaggggaagttttctcaagcaggttgaaagcaggttccaagaaagccctttaaataaacaaggagatagggtgtttattttatggacaagtttcttttgtaacttgtaactcccttgaaagtcagccagagtatgtctcaaaccaaagtcaagatagtgagcaagaagtgttgcacttatgaagggaggtgagtgagcaatgcatgtggtttccaaccgttaatgctagagttatcactttctgttatcaagtggcttcagctatgcaaggaaaccaaacaggggaagttttctcaagcaggttgaaagcaggttccaagaaagccctttagaaatctagctgctacggcttgcgctatggggccgacggcttctctcaaggggcttcgagatgtggcagtgtttaggttgtgtgtaaatgtggttgcattgtcaatagggacgctaaagttcaggccaccttttccatattctctgccagctccctgctcagagatagagcaatttacaccgcttccttcctaccctacccctagcccacccccactctgaaaatttcccaccatcaacggcagaaagcagagaagcagacatcttctagttcctcccccactctcctctttccggtacctgtgagtcagctaggggagggcagctctcacccaggctgatagttcggtgacctggctttatctactggatgagttccgctgggag

SEQ ID NO: 126 - DNA, 430 bp, synthetic construct
  source 1..430: mol_type = other DNA
cccacccagacccctgcctcagggacgcctgtcctcagcccagccctcagctgcagccaggccttcagcctccgtaacccccgctcagggtccccaccccctgcagccctgtccctccaggatgcatggccttgtcctgtgtgggggtggccgagagcactgccccagccctgggtaccttgggcaggaagctggcagaggccagggctgccattcaaacaggggcaggtggttttgccaggaggaagttgacagttcaacttcaaacatgggtgacgcaggccccacactgcctgctccccgtcccacccctccctgagcacgccaccccgccctctccctctctgagagcgagatacccggccagacaccctcacctgcggtgcccagctgcccaggctgaggcaagagaaggccagaaaccatgccc

SEQ ID NO: 127 - DNA, 227 bp, synthetic construct
  source 1..227: mol_type = other DNA
cctattcacgggccccagcctcctcgccgggctggaaggcgacaaccgcgaaaaggagggtgactctcctcggcgggggcttcgggtgacatcacatcctccaaatgcgaaatcaggctccgggccggccgaagggcgcaactttcccccctcggcgccccaccggctcccgcgcgcctcccctcgcgcccgagcttcgagccaagcagcgtcctggggagcgcgtc

SEQ ID NO: 128 - DNA, 967 bp, synthetic construct
  source 1..967: mol_type = other DNA
ggcattcatgcttacccacgggctggtcaacaaagaggtgctgacctgagagtagggcacataacctcagccactggggtacacttaccacccccgcccccgtgtagctccctcccctatcctgaaatctcccttagcacactaagtattctaggttaaacagcccagatgttcagggagttcattcgccaggtgggaagtaatgagatgtaaatcggggtcttttaggtaatagctgacaactggggtaggaatgggggttctgagcccagtgctggctgccgggctgtttatctctgagtcacatcagcaccaagccacagcagccacctgccctagctccatctcttacagtcacaacaggatgtggtttgacatttactgggtcctgcatctggggtgcctgtgaaagttgctccctccacccacccaccttcagagcatcatgagaaccacactcaccgcatccggcacccaaccccctcctatgctgctctttctacctgggcccctggttagcatcctggcagtagaaatagaaggaaagggaaatagggaaagggaaacagggaaagggaaaagaaatctagctgctacggcttgcgctatggggccgacggcttctctcaaggggcttcgagatgtggcagtgtttaggttgtgtgtaaatgtggttgcattgtcaatagggacgctaaagttcaggccaccttttccatattctctgccagctccctgctcagagatagagcaatttacaccgcttccttcctaccctacccctagcccacccccactctgaaaatttcccaccatcaacggcagaaagcagagaagcagacatcttctagttcctcccccactctcctctttccggtacctgtgagtcagctaggggagggcagctctcacccaggctgatagttcggtgacctggctttatctactggatgagttccgctgggag

SEQ ID NO: 129 - protein, 23 aa, synthetic construct
AGTAACTGGTTGAACAACTGTAA

SEQ ID NO: 130 - protein, 21 aa, synthetic construct
CTGGGAGGGAGACGAGGATGA

SEQ ID NO: 131 - DNA, 324 bp, synthetic construct
  source 1..324: mol_type = other DNA
ggcttcccatggtgaatggctggggcgcgtctgtgtccctttctcctctctggctccttgtggcctgaacagccagaaggaagccatgccatgctgtttcagccctcagcttccctcttgcatttcctagaaaagtctttggtgcccagctccagctcagcagattcaggatcccccttcatcatgacttggtcaacgccctgctcaggccaaggtcctctgagagttccaagcttctccactccctataaaaggccggcggaacagccagaggagcagagaggcaaagaaacattgtgaaatctccaactcttaaccttcaac

SEQ ID NO: 132 - DNA, 506 bp, synthetic construct
  source 1..506: mol_type = other DNA
ggggaagatttctcattagatcacgaaaggcctaactgtatataaaagattgaagcatgtgactctcttaaaaggaaaaacaattgtgaaaatccattaaagcattctgctctatcaaaggaggctgtgaccactcatttctgagaaatatctgtcatgtgaaaacataatcacatgattatgcataatcctaagcataatccctgggtgcttccaactcctggtcacccatctggagatacaacttctccataagcccctcaatcaacaagtgaaccactcgtttgtgtaccctaaacctttcaagtaaccataggcaaccctgggctgagaactcacatgacaccaccatagttaaaatgtcttgcatcagcacctccaatgttcccatggtccagtctgcctataaaaaggagagacaacagctcataccccagaaggaggccaggagttgtgagtttccaagccccagctcactctgaccacttctctgcctgcccagcatc

SEQ ID NO: 133 - DNA, 468 bp, synthetic construct
  source 1..468: mol_type = other DNA
cccaggggaagctccgtcttccggcacaggtaatggcctgcagcttgatctccacccagccccatctgagcaggccgggagctcccaggctgtttcacttctctccttcctgactcctcaccatcaccatcgccctctctcctccccaccccgccactcctctcccacacgtgtccctttctccccttcctctgcgtctgctcttctcagaagttagcttacgaagcaaagttgttactttgaattcctgtttttccagccaccctcatgtgacaggatgtctcctcagtagaggctttccctaaattcaggagccctttaaaagggagggcttcctctgtagttcttttcagctgggcagctctgggaacttggattaggtggagaggcagttggggggcctcgttgttttgcgtcttagttccgccctcctgtccatcaggagaaggaaaggataaaccctgggcc

SEQ ID NO: 134 - DNA, 405 bp, synthetic construct
  source 1..405: mol_type = other DNA
catacaaaacaatttcacaaaattgaatgttactcaaaaatcacagctcattttaagctgcacaaaatagtcatttttttctttataattgctcaaattcataatcaaacagaagaaagttcctgtcttggaagtagtgctatgccccaattcttccagagccagtactttaaacaattccatttcattattttcctgtagactaattcttaggacatcagcatatctctcttcaagcattaaaaaaatctctttagagtcagtggatcaatagacagttcctgttttccacacaactgaaagggtggagcccccaaaccacaaggggaagaaggaagttaaaagatgttaaatactggggccagctcaccctggtcagcctagcactctgacctagcagtcaac

SEQ ID NO: 135 - DNA, 438 bp, synthetic construct
  source 1..438: mol_type = other DNA
gcaaactctccaactgtcattgcacagacatatgatctgtatttagctctcactttaggtgtttccattgattctattctcactaatgtgcttcaggtatatccctgtctagaagtcagattggggttaaagagtctgtccgtgattgactaacagtcttaaatacttgatttgttgttgttgttgtcctgtttgtttaagaactttacttctttatccaatgaacggagtatcttgtgtcctggaccctttgcaagaacccttcccctagcaacagatgcgtcatctcaaaatatttttctgattggccaaagagtaattgatttgcattttaatggtcagactctattacaccccacattctcttttcttttattcttgtctgttctgcctcactcccgagctctactgactcccaacagagcgcccaagaagaaa

SEQ ID NO: 136 - DNA, 843 bp, synthetic construct
  source 1..843: mol_type = other DNA
aggactgagctctgagatccttctgaagaggttgggagaagaggagaatcagcaagagaaactgagaaggagggtcatgggcggtaggcgggaagcaggagagtgtggggtcagaggacagatgtagaaatcagttccaggaagcgagggccgagtgtcagaagctgctgctgagtcactcaagatgaagacagaactcatcactggagtcactcaggcagccttggtgaccttgataaaaatagtttaggtggagtaggtgccgggttggagcacaggcttggttggaatggggttaagggaggatgtgagcagtagaacagggtgcagccaacacagacaactactttggagaagttttgcaaaagggaagtaaaaaatgggcagtggttgatgaggagaaacagtttgagagagggcagtggagaagcaagagagctggtctggaacccagctgcctgactcgtgagtcatttctcttcctccaaagccctattaagtctggggctgcttatggtcctcaccaactacacaaagaaagtcagggtcatgctcatccatcaggaggttcagggccacttcccgctttcctctgtttggcaacactaagagtcaccctctgattgttccagaaaagcaagaattgctaaaggccattgtgtcaagtttgcccaattcatgctgcttgacatcttacccctccccaccctgctcccatcccccccacccagtgcccctgattgcaacactcctggctggggtgggacagggtggccagataaaagcagagcaggacctggaaagctggtttgtatgggctgcagcctgccgctgagctgcatc

SEQ ID NO: 137 - DNA, 818 bp, synthetic construct
  source 1..818: mol_type = other DNA
atgtccttcccaggggtgaaagccccctgcctgctgggttcctgccaagactcagctcaaacactaggatgctttggggccccaaggacccagtcacgggactgccccacccgcttcccctctgcggtattaatacgcctcttgctcacttcgggggaaaaacagaaaattgtgcggatgtgggccccagatctgtgggtgtcggttcttctttcagatttgggatcctctgcatgttgggggaggccgcgtctcgctcctcgtttgacctaggtcagaattcaacaggaaggagtttagggtgtccagcaacaacaaccctcaaccatctccagctgagctctcatcccagccccggccctgaccgtaacccgagaaacagtttgagagagggcagtggagaagcaagagagctggtctggaacccagctgcctgactcgtgagtcatttctcttcctccaaagccctattaagtctggggctgcttatggtcctcaccaactacacaaagaaagtcagggtcatgctcatccatcaggaggttcagggccacttcccgctttcctctgtttggcaacactaagagtcaccctctgattgttccagaaaagcaagaattgctaaaggccattgtgtcaagtttgcccaattcatgctgcttgacatcttacccctccccaccctgctcccatcccccccacccagtgcccctgattgcaacactcctggctggggtgggacagggtggccagataaaagcagagcaggacctggaaagctggtttgtatgggctgcagcctgccgctgagctgcatc

SEQ ID NO: 138 - DNA, 782 bp, synthetic construct
  source 1..782: mol_type = other DNA
tagtctcaaaatgcctttcagcataggcaggaaatatgacagaagaaagtcccagtcgaacaaacaataaccgaaaatgctctttgttgctgggccttggcgatcaaagccctgcacatgtttgccagctgtagttcagatggtttctatttcactcagcattaattttttatgaaatctgtggcccaggggcccataagcggcttttagttcttcattctatactgtctggtctaattgccaaggcatggtaagactcagattttaaggtgtcgttaatgtatttaccagccttccggtctacaggcaggctcacctctttgtgtgggattttaatgagaaacagtttgagagagggcagtggagaagcaagagagctggtctggaacccagctgcctgactcgtgagtcatttctcttcctccaaagccctattaagtctggggctgcttatggtcctcaccaactacacaaagaaagtcagggtcatgctcatccatcaggaggttcagggccacttcccgctttcctctgtttggcaacactaagagtcaccctctgattgttccagaaaagcaagaattgctaaaggccattgtgtcaagtttgcccaattcatgctgcttgacatcttacccctccccaccctgctcccatcccccccacccagtgcccctgattgcaacactcctggctggggtgggacagggtggccagataaaagcagagcaggacctggaaagctggtttgtatgggctgcagcctgccgctgagctgcatc

SEQ ID NO: 139 - DNA, 683 bp, synthetic construct
  source 1..683: mol_type = other DNA
agaaagagtgtacttattgaagatgaattgttttcttaatctagtattatcagcctgacagagttattcacaagtagttaagttcctgggaatcacatgagcagcagcaatcccaagaaacctgagtcagtaaaaaaataaattgctgatcttgaagagattcaaagaggaaggcaaaagcattgtcagctttgttcaaactgtatctcaaatttagttgttttttgtttttctatccgagaaacagtttgagagagggcagtggagaagcaagagagctggtctggaacccagctgcctgactcgtgagtcatttctcttcctccaaagccctattaagtctggggctgcttatggtcctcaccaactacacaaagaaagtcagggtcatgctcatccatcaggaggttcagggccacttcccgctttcctctgtttggcaacactaagagtcaccctctgattgttccagaaaagcaagaattgctaaaggccattgtgtcaagtttgcccaattcatgctgcttgacatcttacccctccccaccctgctcccatcccccccacccagtgcccctgattgcaacactcctggctggggtgggacagggtggccagataaaagcagagcaggacctggaaagctggtttgtatgggctgcagcctgccgctgagctgcatc

SEQ ID NO: 140 - DNA, 712 bp, synthetic construct
  source 1..712: mol_type = other DNA
taagaccctaaaagtcacactgtccttagacagttagggaagtagaatggataacatatgcccaaaatacgaatgactaatttccttgcaagatcagctgtctcctgcaagcaacatttgacaattcaccctttcctcgtgatgatgtcttaactaagaagatacaaaaatgcaaggaaatgaaagtgaatatgagatcacttttatgtgctattttaaaaacataaatgcacattgcactgtgtttagggaactatggcttcagaagagaaacagtttgagagagggcagtggagaagcaagagagctggtctggaacccagctgcctgactcgtgagtcatttctcttcctccaaagccctattaagtctggggctgcttatggtcctcaccaactacacaaagaaagtcagggtcatgctcatccatcaggaggttcagggccacttcccgctttcctctgtttggcaacactaagagtcaccctctgattgttccagaaaagcaagaattgctaaaggccattgtgtcaagtttgcccaattcatgctgcttgacatcttacccctccccaccctgctcccatcccccccacccagtgcccctgattgcaacactcctggctggggtgggacagggtggccagataaaagcagagcaggacctggaaagctggtttgtatgggctgcagcctgccgctgagctgcatc

SEQ ID NO: 141 - DNA, 831 bp, synthetic construct
  source 1..831: mol_type = other DNA
aagctgtggcccagaacaccccgatcccactcagaacactatttataagaatgccccgtatgcagtagtctttacagtttttctttttctcaaatgttctttagcctatgtagatgacatttatgcaattcagaggaagatgcctcaacaggattagtcagcagcaaagtcctctgacgcagcttctgtgatctagttaaaaataggaaagaggatgttttgcataagtcatcaccattgtgcggtattggagaattgaccacttttttggttcccacatcctgctaatttatctaaaaatagatgaaaaccctgtccctgaattcctggacaagaccttttgcttctgtgacctcggggctcaggctcttcttgttctgggctccgagaaacagtttgagagagggcagtggagaagcaagagagctggtctggaacccagctgcctgactcgtgagtcatttctcttcctccaaagccctattaagtctggggctgcttatggtcctcaccaactacacaaagaaagtcagggtcatgctcatccatcaggaggttcagggccacttcccgctttcctctgtttggcaacactaagagtcaccctctgattgttccagaaaagcaagaattgctaaaggccattgtgtcaagtttgcccaattcatgctgcttgacatcttacccctccccaccctgctcccatcccccccacccagtgcccctgattgcaacactcctggctggggtgggacagggtggccagataaaagcagagcaggacctggaaagctggtttgtatgggctgcagcctgccgctgagctgcatc

SEQ ID NO: 142 - DNA, 693 bp, synthetic construct
  source 1..693: mol_type = other DNA
agactctgttccctgtatttgcatccactgcctgcgtgctttctctctcccccatatttctgacatttggattttccccctactaattgacatgcctgtcgcctccttctcctggtgtccatttctggaactgctatttgtatattgcatgatattttatcaggaaaaaatataaaacagatctaatttcatgaaaatgctgttgccataatgctcaggagaacagggggaagagagagattcaagtcgagaaacagtttgagagagggcagtggagaagcaagagagctggtctggaacccagctgcctgactcgtgagtcatttctcttcctccaaagccctattaagtctggggctgcttatggtcctcaccaactacacaaagaaagtcagggtcatgctcatccatcaggaggttcagggccacttcccgctttcctctgtttggcaacactaagagtcaccctctgattgttccagaaaagcaagaattgctaaaggccattgtgtcaagtttgcccaattcatgctgcttgacatcttacccctccccaccctgctcccatcccccccacccagtgcccctgattgcaacactcctggctggggtgggacagggtggccagataaaagcagagcaggacctggaaagctggtttgtatgggctgcagcctgccgctgagctgcatc

SEQ ID NO: 143 - DNA, 851 bp, synthetic construct
  source 1..851: mol_type = other DNA
agaaaagagttcacccaataagtttcccaaatttcaaggagcttttgttttattagatgctgttatcttcatgttagtcacaggaaaaaaaaatgcccacatacacacgcacaactaaatgtagtcagtttgctcagctgctgctgacgtcactgctgcccactaggagtgagttactgtcataacccctcttttattaatcataggctggaggaagcacaaagtgagtgacatcattaggcaaaggaccggctaactcatgctccaatttactcagctttattataacatttctcgagtgtcatatgaaagtgattaccatttcacactttccccatctgagcaatcatccctaaccttcaattcaaattcccagagaaaagcttagcttttcagatggaggtgcgagaaacagtttgagagagggcagtggagaagcaagagagctggtctggaacccagctgcctgactcgtgagtcatttctcttcctccaaagccctattaagtctggggctgcttatggtcctcaccaactacacaaagaaagtcagggtcatgctcatccatcaggaggttcagggccacttcccgctttcctctgtttggcaacactaagagtcaccctctgattgttccagaaaagcaagaattgctaaaggccattgtgtcaagtttgcccaattcatgctgcttgacatcttacccctccccaccctgctcccatcccccccacccagtgcccctgattgcaacactcctggctggggtgggacagggtggccagataaaagcagagcaggacctggaaagctggtttgtatgggctgcagcctgccgctgagctgcatc

SEQ ID NO: 144 - DNA, 826 bp, synthetic construct
  source 1..826: mol_type = other DNA
ttctttcagcaaaacctttcggagaagcccaatactaagctcctctggttagagccagccatgagagaaactccaagtacttctgactggttctctctctactcatccaccccttaggtggctgcagaaggaactctgtgcaacccccagagttctcattctcagtgacagggaaatgtaatgattggccctggatgattcagcagatcagatgatacttactcagagcaatttccactcctttgcagtagcatattatcagtattttccagataaataacttggctaaagaaaaatccatttcatttacatctttggcaccttacagcaatagaacttttgtgcaatgattttaatattatatttctacattggctgatagagaaacagtttgagagagggcagtggagaagcaagagagctggtctggaacccagctgcctgactcgtgagtcatttctcttcctccaaagccctattaagtctggggctgcttatggtcctcaccaactacacaaagaaagtcagggtcatgctcatccatcaggaggttcagggccacttcccgctttcctctgtttggcaacactaagagtcaccctctgattgttccagaaaagcaagaattgctaaaggccattgtgtcaagtttgcccaattcatgctgcttgacatcttacccctccccaccctgctcccatcccccccacccagtgcccctgattgcaacactcctggctggggtgggacagggtggccagataaaagcagagcaggacctggaaagctggtttgtatgggctgcagcctgccgctgagctgcatc

SEQ ID NO: 145 - DNA, 901 bp, synthetic construct
  source 1..901: mol_type = other DNA
gaaatcctcgaaatgagatactgtcccgtgattctgagagtgacccaaaaggatacggaatgaggtactaaaagcaggtgcttggaaacctgagggcagtggtgttcatgcgtttcccggcactttgactttcagcctcctgcaagcctctccttctttgccttcctgaccgttagatacaattaatttggggtttgttttttctgcttcctctttcccctcccaccctatgtttcagttctaaagttagaaggtcctctcatccttttaagaagaacagagacagaaaatggttagtcaccatctaggacagactacaattccagatcattgcaggacgtgcccactcaaatggatgattattgagagctggccacctgaagtgttttacacaggcagtgatctaagggttgaagctatctggcctttttgcttgcttgttatgtatttatggctgagaaacagtttgagagagggcagtggagaagcaagagagctggtctggaacccagctgcctgactcgtgagtcatttctcttcctccaaagccctattaagtctggggctgcttatggtcctcaccaactacacaaagaaagtcagggtcatgctcatccatcaggaggttcagggccacttcccgctttcctctgtttggcaacactaagagtcaccctctgattgttccagaaaagcaagaattgctaaaggccattgtgtcaagtttgcccaattcatgctgcttgacatcttacccctccccaccctgctcccatcccccccacccagtgcccctgattgcaacactcctggctggggtgggacagggtggccagataaaagcagagcaggacctggaaagctggtttgtatgggctgcagcctgccgctgagctgcatc

SEQ ID NO: 146 - DNA, 633 bp, synthetic construct
  source 1..633: mol_type = other DNA
ccctagctctggggaaatgaaagccaggctggggttcaaatgagggcagtttcccttcctgtgggctgctgatggaacaaccccatgacgagaaggacccagcctccaagcggccacaccctgtgtgtctctttgtcctgccggcactgaggactcatccatctgcacagctggggcccctgggaggagagaaacagtttgagagagggcagtggagaagcaagagagctggtctggaacccagctgcctgactcgtgagtcatttctcttcctccaaagccctattaagtctggggctgcttatggtcctcaccaactacacaaagaaagtcagggtcatgctcatccatcaggaggttcagggccacttcccgctttcctctgtttggcaacactaagagtcaccctctgattgttccagaaaagcaagaattgctaaaggccattgtgtcaagtttgcccaattcatgctgcttgacatcttacccctccccaccctgctcccatcccccccacccagtgcccctgattgcaacactcctggctggggtgggacagggtggccagataaaagcagagcaggacctggaaagctggtttgtatgggctgcagcctgccgctgagctgcatc

SEQ ID NO: 147 - DNA, 1017 bp, synthetic construct
  source 1..1017: mol_type = other DNA
cgtcccggtcccggccgggcctgggactctccgcgccccggtggggcctgaagctccgggtaccgccgagtcctcccctactggcggctgggggagggaacgagggcggggctctcggaaagtcccaggaacaggctgatcctgcgctggcgagaagctcagccatttaggggaaagcgaaatcgaaagcggccgcctgctcactagataacgcctacttccaaaagtggcctgcccagactattttggtagcaagcgtggaaatcagatctgagaatctcgggagcagccctggtgcccaattttctccatcacgcacacccttctcgcctctccctgcctcctgcctttccacttgcaccagttttcccaccccagcctcagggcggggctgcctcgtcacttgtctcggggcagatctgccctacacacgttagcgccgcgcgcaaagcagccccgcagcacccaggcgcctcctggcggcgccgcgaaggggcggggctgtcggctgcgcgttgtgcgctgtcccaggttggaaaccagtgccccaggcggcgaggagagcggtgcctgagaaacagtttgagagagggcagtggagaagcaagagagctggtctggaacccagctgcctgactcgtgagtcatttctcttcctccaaagccctattaagtctggggctgcttatggtcctcaccaactacacaaagaaagtcagggtcatgctcatccatcaggaggttcagggccacttcccgctttcctctgtttggcaacactaagagtcaccctctgattgttccagaaaagcaagaattgctaaaggccattgtgtcaagtttgcccaattcatgctgcttgacatcttacccctccccaccctgctcccatcccccccacccagtgcccctgattgcaacactcctggctggggtgggacagggtggccagataaaagcagagcaggacctggaaagctggtttgtatgggctgcagcctgccgctgagctgcatc

SEQ ID NO: 148 - DNA, 824 bp, synthetic construct
  source 1..824: mol_type = other DNA
aaggcggcgccagggagagggcgcagtctctgaatctttccacggggtccatcctagggcccctccaggttcaacggtctcctaacctgtagtcacccacaagagcgtgccctttctgcccgcccttcctagcgttgctccctgcttggctgagcactgcggagtttcacgcctctaaaccccgcctcttcttgcaacctgtgttggcctcatctacccagcaactgtcgacgtcacacgacctgggcctccctgaatgggagatatttactaggcaatcccgcctactgttctgaggtttcccctccaggtgcagcttcagagccaggcgagccaggaaggaccagcgggcgaggtggtgagttgtgaggcgcgcccagagaaacagtttgagagagggcagtggagaagcaagagagctggtctggaacccagctgcctgactcgtgagtcatttctcttcctccaaagccctattaagtctggggctgcttatggtcctcaccaactacacaaagaaagtcagggtcatgctcatccatcaggaggttcagggccacttcccgctttcctctgtttggcaacactaagagtcaccctctgattgttccagaaaagcaagaattgctaaaggccattgtgtcaagtttgcccaattcatgctgcttgacatcttacccctccccaccctgctcccatcccccccacccagtgcccctgattgcaacactcctggctggggtgggacagggtggccagataaaagcagagcaggacctggaaagctggtttgtatgggctgcagcctgccgctgagctgcatc

SEQ ID NO: 149 - DNA, 894 bp, synthetic construct
  source 1..894: mol_type = other DNA
cttctgcccgacccgaggtacctccaccctgtctaccaggttcagccccgccctctcatcatgtattggcccccaaaacgcggctcttccctcccatcagtttgtctttccactctcattggtcctcaggacgaccgtgactccgcccacctacaccacatttccaccactatccctgacttccaatggccccgccccagccactaaggttcggccttttctgcccagctggccgcctcttccttggtctggtgtcccaggcaccgcccacgggtctagcctcttctcaggagtgctctacagcgccccctaggccaccaagattgtttagctccctgtcgggtcggcccctgactccttattggactcatccatctggctcatccaaggccttgggtctctccagctgactcgacggtgatggggggcaactcggcgggggagctgtggagaaacagtttgagagagggcagtggagaagcaagagagctggtctggaacccagctgcctgactcgtgagtcatttctcttcctccaaagccctattaagtctggggctgcttatggtcctcaccaactacacaaagaaagtcagggtcatgctcatccatcaggaggttcagggccacttcccgctttcctctgtttggcaacactaagagtcaccctctgattgttccagaaaagcaagaattgctaaaggccattgtgtcaagtttgcccaattcatgctgcttgacatcttacccctccccaccctgctcccatcccccccacccagtgcccctgattgcaacactcctggctggggtgggacagggtggccagataaaagcagagcaggacctggaaagctggtttgtatgggctgcagcctgccgctgagctgcatc

SEQ ID NO: 150 - DNA, 1092 bp, synthetic construct
  source 1..1092: mol_type = other DNA
gattacagcagaggcctctttgtcagtgccagtaccgtctcctcttagccaccctggggatggggctcattattattgcttggcagatgagaagcaggaggctcagagaaggtaaataacttgcccgaatttacacgcagccagtaaatggccaagccagaatttaaaccagcttttctgactccaaatctagtgctctttttaccacaccacagctgcctcaggctagggcaggacatcaacaaataaaaatgaatcgtctagactcaatacaaacagggaagaagaaaagtgggacagggggaggatgtagtgctggccaaacccagggctgaaatccagacttccccaagtgtggtaaggcaaggcaaggcaagcaagagatgtctccaggggctggggctcgtcagtggaagatcggaaacctaagcatgcaagagattgcaacacacggccttagatgagagaaacagccttgaaacagaccacggagaaaagaaggagaacatgaaaatgccacctcccccagttgtataagacctgcccagatacccccctggagccattcccaaggatctctccagacctaagcaagtcccagggcctaccctgccttcccagatcatctcctctctgtgggactcacagagaaacagtttgagagagggcagtggagaagcaagagagctggtctggaacccagctgcctgactcgtgagtcatttctcttcctccaaagccctattaagtctggggctgcttatggtcctcaccaactacacaaagaaagtcagggtcatgctcatccatcaggaggttcagggccacttcccgctttcctctgtttggcaacactaagagtcaccctctgattgttccagaaaagcaagaattgctaaaggccattgtgtcaagtttgcccaattcatgctgcttgacatcttacccctccccaccctgctcccatcccccccacccagtgcccctgattgcaacactcctggctggggtgggacagggtggccagataaaagcagagcaggacctggaaagctggtttgtatgggctgcagcctgccgctgagctgcatc

SEQ ID NO: 151 - DNA, 1000 bp, synthetic construct
  source 1..1000: mol_type = other DNA
cctagctcttagtgtaatgattatgggaacagggtcaaatagcaaatcacaaattatttcacgactattgtgagacaagagtgagagccaagagtggtggtgcacacctgtaatcccagctcgaaccagggagacagaggttgcagtgagccgagatcgcaccaatggcttaacacaatgggatttggcttttcactcatgtaaatgaccagtgcggttttctctggggcagaatttgaattttctccccaggatgactcagggacacccgcttcctccattgtgctcccatcatgcccttgggcaatggcgtcccgtacttcaaacagcaagaaagaaggagaaacagaatatatctgtgcacttgcaaaatttgctgacacatgtcatttctgtccagaattgttggctataaatagtgttatgaacagtcacacaatgatgcaacaagaccagggaaaaagtcccttggtgggggtagccacttcccagaggttccaatgcttgcactgtaagggtaagtacagaattttttttttttctggtgagcagccagagaaacagtttgagagagggcagtggagaagcaagagagctggtctggaacccagctgcctgactcgtgagtcatttctcttcctccaaagccctattaagtctggggctgcttatggtcctcaccaactacacaaagaaagtcagggtcatgctcatccatcaggaggttcagggccacttcccgctttcctctgtttggcaacactaagagtcaccctctgattgttccagaaaagcaagaattgctaaaggccattgtgtcaagtttgcccaattcatgctgcttgacatcttacccctccccaccctgctcccatcccccccacccagtgcccctgattgcaacactcctggctggggtgggacagggtggccagataaaagcagagcaggacctggaaagctggtttgtatgggctgcagcctgccgctgagctgcatc

SEQ ID NO: 152 - DNA, 964 bp, synthetic construct
  source 1..964: mol_type = other DNA
ttattactctatagataaagcagagtctctgaagttaactaacttccccaaagtcacacatcgtggaaccatgaatcttaccaggttctgtgtgactccaaatttgtgctctttcatattgcacaacactgtccagattaattcaagtggagagtgaactttttctggtacatcccttagtctcttgcacagccattgcctttcacacacccagactgtttctttgctttagggactggaaagtggaagtggaaccccctatgttctgtcctgggatatttccggggtgagccaagagtagctgtgtgtcctgctaggtcatggactttcactgaccacagaagttgagaacccttgagcaaactaaattcttatatcttactggtttgggagcaaagcagaagtggcaaaagctgacaaaacccagctggagcaggaatgttgaaatggacacaaataaacataccctgtggacacaatcaatataaatgttctaaatttacttctgctcctatgcttgagaaacagtttgagagagggcagtggagaagcaagagagctggtctggaacccagctgcctgactcgtgagtcatttctcttcctccaaagccctattaagtctggggctgcttatggtcctcaccaactacacaaagaaagtcagggtcatgctcatccatcaggaggttcagggccacttcccgctttcctctgtttggcaacactaagagtcaccctctgattgttccagaaaagcaagaattgctaaaggccattgtgtcaagtttgcccaattcatgctgcttgacatcttacccctccccaccctgctcccatcccccccacccagtgcccctgattgcaacactcctggctggggtgggacagggtggccagataaaagcagagcaggacctggaaagctggtttgtatgggctgcagcctgccgctgagctgcatc

SEQ ID NO: 153 - DNA, 814 bp, synthetic construct
  source 1..814: mol_type = other DNA
aaaaagtgttaaatcgtccaaaaaggaggaaagaaaggggaaaaaaagtaacaattctaaatctttatgtgcctgataacacggcttcaacacatcgaataaaatgtttacagaactgtaagtagaatcgcagcggaagatttcaacacaattcttttcatatggaaagaggaagaagcacgtaaaaatcacagaactacaagcacgtggagcatgttctctgatcacagtggaactaagcctgaaacctaaaacaaagagataaccagaaacacatatgtttgtaaattaagaaatgcatttctaaataactcctgggtcaaagagcagctcacagtggaaatcagaaagtattttgaactgaaagacgagaaacagtttgagagagggcagtggagaagcaagagagctggtctggaacccagctgcctgactcgtgagtcatttctcttcctccaaagccctattaagtctggggctgcttatggtcctcaccaactacacaaagaaagtcagggtcatgctcatccatcaggaggttcagggccacttcccgctttcctctgtttggcaacactaagagtcaccctctgattgttccagaaaagcaagaattgctaaaggccattgtgtcaagtttgcccaattcatgctgcttgacatcttacccctccccaccctgctcccatcccccccacccagtgcccctgattgcaacactcctggctggggtgggacagggtggccagataaaagcagagcaggacctggaaagctggtttgtatgggctgcagcctgccgctgagctgcatc

SEQ ID NO: 154 - protein, 361 aa, synthetic construct
KFTIVFPHNQKGNWKNVPSNYHYCPSSSDLNWHNDLIGTALQVKMPKSHKARQADGWMCHASKWVTTCDFRWYGPKYITHSIRSFTPSVEQCKESIEQTKQGTWLNPGFPPQSCGYATVTDAEAVIVQVTPHHVLVDEYTGEWVDSQFINGKCSNYICPTVHNSTTWHSDYKVKGLCDSNLISMDITFFSEDGELSSLGKEGTGFRSNYFAYETGGKACKMQYCKHWGVRLPSGVWFEMADKDLFAAARFPECPEGSSISAPSQTSVDVSLIQDVERILDYSLCQETWSKIRAGLPISPVDLSYLAPKNPGTGPAFTIINGTLKYFETRYERVDIAAPILSRMVGMISGTTTERLLWDDWA

SEQ ID NO: 155 - protein, 361 aa, synthetic construct
KFTIVFPHQQKGNWKNVPSNYHYCPSSSDLNWHNDLIGTALQVKMPKVHKAIQADGWMCHASKWVTTCDFRWYGPKYITHSIRSFTPSVEQCKESIEQTKQGTWLNPGFPPQSCGYATVTDAEAVIVQVTPHHVLVDEYTGEWVDSQFINGKCSNYICPTVHNSTTWHSDYKVKGLCDSNLISMDITFFSEDGELSSLGKEGTGFRSNYFAYETGGKACKMQYCKHWGVRLPSGVWFEMADKDLFAAARFPECPEGSSISAPSQTSVDVSLIQDVERILDYSLCQETWSKIRAGLPISPVDLSYLAPKNPGTGPAFTIINGTLKYFETRYIRIDIAAPILSRMVGMISGTTTKRELWDDWA

SEQ ID NO: 156 - protein, 361 aa, synthetic construct
KFTIVFPHGQKGNWKNVPSNYHYCPSSSDLNWHNDLIGTALQVKMPGSHKAIQADGWMCHASKWVTTCDFRWYGPKYITHSIRSFTPSVEQCKESIEQTKQGTWLNPGFPPQSCGYATVTDAEAVIVQVTPHHVLVDEYTGEWVDSQFINGKCSNYICPTVHNSTTWHSDYKVKGLCDSNLISMDITFFSEDGELSSLGKEGTGFRSNYFAYETGGKACKMQYCKHWGVRLPSGVWFEMADKDLFAAARFPECPEGSSISAPSQTSVDVSLIQDVERILDYSLCQETWSKIRAGLPISPVDLSYLAPKNPGTGPAFTIINGTLKYFETRYERVDIAAPILSRMVGMISGTTSERELWDDWA

SEQ ID NO: 157 - protein, 361 aa, synthetic construct
KFTIVFPFNQKGNWKNVPSNYHYCPSSSDLNWHNDLIGTALQVKMPKSHKPIQADGWMCHASKWVTTCDFRWYGPKYITHSIRSFTPSVEQCKESIEQTKQGTWLNPGFPPQSCGYATVTDAEAVIVQVTPHHVLVDEYTGEWVDSQFINGKCSNYICPTVHNSTTWHSDYKVKGLCDSNLISMDITFFSEDGELSSLGKEGTGFRSNYFAYETGGKACKMQYCKHWGVRLPSGVWFEMADKDLFAAARFPECPEGSSISAPSQTSVDVSLIQDVERILDYSLCQETWSKIRAGLPISPVDLSYLAPKNPGTGPAFTIINGTLKYFETVYIRVDIAAPILSRMVGMISGTTVERELWDDWA

SEQ ID NO: 158 - protein, 361 aa, synthetic construct
KFTIVFPHQQKGNWKNVPSNYHYCPSSSDLNWHNDLIGTALQVKMPTSHKAIQADGWMCHASKWVTTCDFRWYGPKYITHSIRSFTPSVEQCKESIEQTKQGTWLNPGFPPQSCGYATVTDAEAVIVQVTPHHVLVDEYTGEWVDSQFINGKCSNYICPTVHNSTTWHSDYKVKGLCDSNLISMDITFFSEDGELSSLGKEGTGFRSNYFAYETGGKACKMQYCKHWGVRLPSGVWFEMADKDLFAAARFPECPEGSSISAPSQTSVDVSLIQDVERILDYSLCQETWSKIRAGLPISPVDLSYLAPKNPGTGPAFTIINGTLKYFESRYIRVDIAAPILSRMVGMISGTTTERLLWDDWA

SEQ ID NO: 159 - protein, 361 aa, synthetic construct
KFTIVFPHGQKGNWKNVPSNYHYCPSSSDLNWHNDLIGTALQVKMPKSHSAIQADGWMCHASKWVTTCDFRWYGPKYITHSIRSFTPSVEQCKESIEQTKQGTWLNPGFPPQSCGYATVTDAEAVIVQVTPHHVLVDEYTGEWVDSQFINGKCSNYICPTVHNSTTWHSDYKVKGLCDSNLISMDITFFSEDGELSSLGKEGTGFRSNYFAYETGGKACKMQYCKHWGVRLPSGVWFEMADKDLFAAARFPECPEGSSISAPSQTSVDVSLIQDVERILDYSLCQETWSKIRAGLPISPVDLSYLAPKNPGTGPAFTIINGTLKYFETRYIRIDIAAPILSRMVGMISGTRTERELWDDWA

SEQ ID NO: 160 - protein, 361 aa, synthetic construct
KFTIVFPFNQKGNWKNVPSNYHYCPSSSDLNWHNDLIGTALQVKMPKLHKAIQADGWMCHASKWVTTCDFRWYGPKYITHSIRSFTPSVEQCKESIEQTKQGTWLNPGFPPQSCGYATVTDAEAVIVQVTPHHVLVDEYTGEWVDSQFINGKCSNYICPTVHNSTTWHSDYKVKGLCDSNLISMDITFFSEDGELSSLGKEGTGFRSNYFAYETGGKACKMQYCKHWGVRLPSGVWFEMADKDLFAAARFPECPEGSSISAPSQTSVDVSLIQDVERILDYSLCQETWSKIRAGLPISPVDLSYLAPKNPGTGPAFTIINGTLKYFETKYIRVDIAAPILSRMVGMISGTTTERELWDDWA

SEQ ID NO: 161 - protein, 361 aa, synthetic construct
KFTIVFPYNQKGNWKNVPSNYHYCPSSSDLNWHNDLIGTALQVKMPGSHKAIQADGWMCHASKWVTTCDFRWYGPKYITHSIRSFTPSVEQCKESIEQTKQGTWLNPGFPPQSCGYATVTDAEAVIVQVTPHHVLVDEYTGEWVDSQFINGKCSNYICPTVHNSTTWHSDYKVKGLCDSNLISMDITFFSEDGELSSLGKEGTGFRSNYFAYETGGKACKMQYCKHWGVRLPSGVWFEMADKDLFAAARFPECPEGSSISAPSQTSVDVSLIQDVERILDYSLCQETWSKIRAGLPISPVDLSYLAPKNPGTGPAFTIINGTLKYFETRYIRVDIAAPILSRMVGMISGTTTERELWDDWA

SEQ ID NO: 162 - protein, 361 aa, synthetic construct
KFTIVFPHHQKGNWKNVPSNYHYCPSSSDLNWHNDLIGTALQVKMPKRHKAIQADGWMCHASKWVTTCDFRWYGPKYITHSIRSFTPSVEQCKESIEQTKQGTWLNPGFPPQSCGYATVTDAEAVIVQVTPHHVLVDEYTGEWVDSQFINGKCSNYICPTVHNSTTWHSDYKVKGLCDSNLISMDITFFSEDGELSSLGKEGTGFRSNYFAYETGGKACKMQYCKHWGVRLPSGVWFEMADKDLFAAARFPECPEGSSISAPSQTSVDVSLIQDVERILDYSLCQETWSKIRAGLPISPVDLSYLAPKNPGTGPAFTIINGTLKYFETRYIRVDIAAPILSRMVGMISGTTEERELWDDWA

SEQ ID NO: 163 - protein, 361 aa, synthetic construct
KFTIVFPHGQKGNWKNVPSNYHYCPSSSDLNWHNDLIGTALQVKMPKSFKAIQADGWMCHASKWVTTCDFRWYGPKYITHSIRSFTPSVEQCKESIEQTKQGTWLNPGFPPQSCGYATVTDAEAVIVQVTPHHVLVDEYTGEWVDSQFINGKCSNYICPTVHNSTTWHSDYKVKGLCDSNLISMDITFFSEDGELSSLGKEGTGFRSNYFAYETGGKACKMQYCKHWGVRLPSGVWFEMADKDLFAAARFPECPEGSSISAPSQTSVDVSLIQDVERILDYSLCQETWSKIRAGLPISPVDLSYLAPKNPGTGPAFTIINGTLKYFETTYIRVDIAAPILSRMVGMISGGTTERELWDDWA

SEQ ID NO: 164 - protein, 361 aa, synthetic construct
KFTIVFPLNQKGNWKNVPSNYHYCPSSSDLNWHNDLIGTALQVKLPKSHKAIQADGWMCHASKWVTTCDFRWYGPKYITHSIRSFTPSVEQCKESIEQTKQGTWLNPGFPPQSCGYATVTDAEAVIVQVTPHHVLVDEYTGEWVDSQFINGKCSNYICPTVHNSTTWHSDYKVKGLCDSNLISMDITFFSEDGELSSLGKEGTGFRSNYFAYETGGKACKMQYCKHWGVRLPSGVWFEMADKDLFAAARFPECPEGSSISAPSQTSVDVSLIQDVERILDYSLCQETWSKIRAGLPISPVDLSYLAPKNPGTGPAFTIINGTLKYFETRYERVDIAAPILSRMVGMISGTTTERRLWDDWA

SEQ ID NO: 165 - protein, 361 aa, synthetic construct
KFTIVFPHNQEGNWKNVPSNYHYCPSSSDLNWHNDLIGTALQVKMPKFHKAIQADGWMCHASKWVTTCDFRWYGPKYITHSIRSFTPSVEQCKESIEQTKQGTWLNPGFPPQSCGYATVTDAEAVIVQVTPHHVLVDEYTGEWVDSQFINGKCSNYICPTVHNSTTWHSDYKVKGLCDSNLISMDITFFSEDGELSSLGKEGTGFRSNYFAYETGGKACKMQYCKHWGVRLPSGVWFEMADKDLFAAARFPECPEGSSISAPSQTSVDVSLIQDVERILDYSLCQETWSKIRAGLPISPVDLSYLAPKNPGTGPAFTIINGTLKYFETRLIRVDIAAPILSRMVGMISGTTDERELWDDWA

SEQ ID NO: 166 - protein, 361 aa, synthetic construct
KFTIVFPHDQKGNWKNVPSNYHYCPSSSDLNWHNDLIGTALQVKMPKSHKSIQADGWMCHASKWVTTCDFRWYGPKYITHSIRSFTPSVEQCKESIEQTKQGTWLNPGFPPQSCGYATVTDAEAVIVQVTPHHVLVDEYTGEWVDSQFINGKCSNYICPTVHNSTTWHSDYKVKGLCDSNLISMDITFFSEDGELSSLGKEGTGFRSNYFAYETGGKACKMQYCKHWGVRLPSGVWFEMADKDLFAAARFPECPEGSSISAPSQTSVDVSLIQDVERILDYSLCQETWSKIRAGLPISPVDLSYLAPKNPGTGPAFTIINGTLKYFETRYTRVDIAAPILSRMVGMISGTTTERHLWDDWA

SEQ ID NO: 167 - protein, 361 aa, synthetic construct
KFTIVFPHNQKGNWKNVPSNYHYCPSSSDLNWHNDLIGTALQVKMPKSHKTIQADGWMCHASKWVTTCDFRWYGPKYITHSIRSFTPSVEQCKESIEQTKQGTWLNPGFPPQSCGYATVTDAEAVIVQVTPHHVLVDEYTGEWVDSQFINGKCSNYICPTVHNSTTWHSDYKVKGLCDSNLISMDITFFSEDGELSSLGKEGTGFRSNYFAYETGGKACKMQYCKHWGVRLPSGVWFEMADKDLFAAARFPECPEGSSISAPSQTSVDVSLIQDVERILDYSLCQETWSKIRAGLPISPVDLSYLAPKNPGTGPAFTIINGTLKYFETWYIRVDIAAPILSRMVGMISGTTTERELWDDWA

SEQ ID NO: 168 - protein, 361 aa, synthetic construct
KFTIVFPHNVKGNWKNVPSNYHYCPSSSDLNWHNDLIGTALQVKMPKSHKAIAADGWMCHASKWVTTCDFRWYGPKYITHSIRSFTPSVEQCKESIEQTKQGTWLNPGFPPQSCGYATVTDAEAVIVQVTPHHVLVDEYTGEWVDSQFINGKCSNYICPTVHNSTTWHSDYKVKGLCDSNLISMDITFFSEDGELSSLGKEGTGFRSNYFAYETGGKACKMQYCKHWGVRLPSGVWFEMADKDLFAAARFPECPEGSSISAPSQTSVDVSLIQDVERILDYSLCQETWSKIRAGLPISPVDLSYLAPKNPGTGPAFTIINGTLKYFETRYERVDIAAPILSRMVGMISGTTIERELWDDWA

SEQ ID NO: 169 - protein, 361 aa, synthetic construct
KFTIVRPHNKKGNWKNVPSNYHYCPSSSDLNWHNDLIGTALQVKMPKSHTAIQADGWMCHASKWVTTCDFRWYGPKYITHSIRSFTPSVEQCKESIEQTKQGTWLNPGFPPQSCGYATVTDAEAVIVQVTPHHVLVDEYTGEWVDSQFINGKCSNYICPTVHNSTTWHSDYKVKGLCDSNLISMDITFFSEDGELSSLGKEGTGFRSNYFAYETGGKACKMQYCKHWGVRLPSGVWFEMADKDLFAAARFPECPEGSSISAPSQTSVDVSLIQDVERILDYSLCQETWSKIRAGLPISPVDLSYLAPKNPGTGPAFTIINGTLKYFETRYIRPDIAAPILSRMVGMISGTTRERELWDDWA

SEQ ID NO: 170 - protein, 361 aa, synthetic construct
KFTIVFPHNQKGNWKNVPSNYHYCPSSSDLNWHNDLIGTALQVKMPKMHKAIQADGWMCHASKWVTTCDFRWYGPKYITHSIRSFTPSVEQCKESIEQTKQGTWLNPGFPPQSCGYATVTDAEAVIVQVTPHHVLVDEYTGEWVDSQFINGKCSNYICPTVHNSTTWHSDYKVKGLCDSNLISMDITFFSEDGELSSLGKEGTGFRSNYFAYETGGKACKMQYCKHWGVRLPSGVWFEMADKDLFAAARFPECPEGSSISAPSQTSVDVSLIQDVERILDYSLCQETWSKIRAGLPISPVDLSYLAPKNPGTGPAFTIINGTLKYFETRPIRVDIAAPILSRMVGMISGTDTERELWDDWA

SEQ ID NO: 171 - protein, 361 aa, synthetic construct
KFTIVFPHTQKGNWKNVPSNYHYCPSSSDLNWHNDLIGTALQVKMPKSHKATQADGWMCHASKWVTTCDFRWYGPKYITHSIRSFTPSVEQCKESIEQTKQGTWLNPGFPPQSCGYATVTDAEAVIVQVTPHHVLVDEYTGEWVDSQFINGKCSNYICPTVHNSTTWHSDYKVKGLCDSNLISMDITFFSEDGELSSLGKEGTGFRSNYFAYETGGKACKMQYCKHWGVRLPSGVWFEMADKDLFAAARFPECPEGSSISAPSQTSVDVSLIQDVERILDYSLCQETWSKIRAGLPISPVDLSYLAPKNPGTGPAFTIINGTLKYFETKYIRVDIAAPILSRMVGMISGTTEERELWDDWA

SEQ ID NO: 172 - protein, 361 aa, synthetic construct
KFTIVIPHNQKGNWKNVPSNYHYCPSSSDLNWHNDLIGTALQVKMPVSHKAIQADGWMCHASKWVTTCDFRWYGPKYITHSIRSFTPSVEQCKESIEQTKQGTWLNPGFPPQSCGYATVTDAEAVIVQVTPHHVLVDEYTGEWVDSQFINGKCSNYICPTVHNSTTWHSDYKVKGLCDSNLISMDITFFSEDGELSSLGKEGTGFRSNYFAYETGGKACKMQYCKHWGVRLPSGVWFEMADKDLFAAARFPECPEGSSISAPSQTSVDVSLIQDVERILDYSLCQETWSKIRAGLPISPVDLSYLAPKNPGTGPAFTIINGTLKYFETRYIRVAIAAPILSRMVGMISGTTTEDELWDDWA

SEQ ID NO: 173 - protein, 361 aa, synthetic construct
KFTIVFPSNQKGNWKNVPSNYHYCPSSSDLNWHNDLIGTALQVKMPKSAKAIQADGWMCHASKWVTTCDFRWYGPKYITHSIRSFTPSVEQCKESIEQTKQGTWLNPGFPPQSCGYATVTDAEAVIVQVTPHHVLVDEYTGEWVDSQFINGKCSNYICPTVHNSTTWHSDYKVKGLCDSNLISMDITFFSEDGELSSLGKEGTGFRSNYFAYETGGKACKMQYCKHWGVRLPSGVWFEMADKDLFAAARFPECPEGSSISAPSQTSVDVSLIQDVERILDYSLCQETWSKIRAGLPISPVDLSYLAPKNPGTGPAFTIINGTLKYFETHYIRVDIAAPILSRMVGMISGTTQERELWDDWA

SEQ ID NO: 174 - protein, 361 aa, synthetic construct
KFTIVFPHNQAGNWKNVPSNYHYCPSSSDLNWHNDLIGTALQVKMPKLHKAIQADGWMCHASKWVTTCDFRWYGPKYITHSIRSFTPSVEQCKESIEQTKQGTWLNPGFPPQSCGYATVTDAEAVIVQVTPHHVLVDEYTGEWVDSQFINGKCSNYICPTVHNSTTWHSDYKVKGLCDSNLISMDITFFSEDGELSSLGKEGTGFRSNYFAYETGGKACKMQYCKHWGVRLPSGVWFEMADKDLFAAARFPECPEGSSISAPSQTSVDVSLIQDVERILDYSLCQETWSKIRAGLPISPVDLSYLAPKNPGTGPAFTIINGTLKYFETRYLRVDIAAPILSRMVGMISGTTTEKELWDDWA

SEQ ID NO: 175 - protein, 361 aa, synthetic construct
KFTIVFWHNQKGNWKNVPSNYHYCPSSSDLNWHNDLIGTALQVKFPKSHKAIQADGWMCHASKWVTTCDFRWYGPKYITHSIRSFTPSVEQCKESIEQTKQGTWLNPGFPPQSCGYATVTDAEAVIVQVTPHHVLVDEYTGEWVDSQFINGKCSNYICPTVHNSTTWHSDYKVKGLCDSNLISMDITFFSEDGELSSLGKEGTGFRSNYFAYETGGKACKMQYCKHWGVRLPSGVWFEMADKDLFAAARFPECPEGSSISAPSQTSVDVSLIQDVERILDYSLCQETWSKIRAGLPISPVDLSYLAPKNPGTGPAFTIINGTLKYFETRYIRYDIAAPILSRMVGMISGTTTEVELWDDWA

SEQ ID NO: 176 - protein, 361 aa, synthetic construct
KFTIVFPHRQKGNWKNVPSNYHYCPSSSDLNWHNDLIGTALQVKMPKSHKAIIADGWMCHASKWVTTCDFRWYGPKYITHSIRSFTPSVEQCKESIEQTKQGTWLNPGFPPQSCGYATVTDAEAVIVQVTPHHVLVDEYTGEWVDSQFINGKCSNYICPTVHNSTTWHSDYKVKGLCDSNLISMDITFFSEDGELSSLGKEGTGFRSNYFAYETGGKACKMQYCKHWGVRLPSGVWFEMADKDLFAAARFPECPEGSSISAPSQTSVDVSLIQDVERILDYSLCQETWSKIRAGLPISPVDLSYLAPKNPGTGPAFTIINGTLKYFETRYQRVDIAAPILSRMVGMISGTTTEMELWDDWA

SEQ ID NO: 177 - protein, 361 aa, synthetic construct
KFTIVFPSNQKGNWKNVPSNYHYCPSSSDLNWHNDLIGTALQVKMPKSHKAVQADGWMCHASKWVTTCDFRWYGPKYITHSIRSFTPSVEQCKESIEQTKQGTWLNPGFPPQSCGYATVTDAEAVIVQVTPHHVLVDEYTGEWVDSQFINGKCSNYICPTVHNSTTWHSDYKVKGLCDSNLISMDITFFSEDGELSSLGKEGTGFRSNYFAYETGGKACKMQYCKHWGVRLPSGVWFEMADKDLFAAARFPECPEGSSISAPSQTSVDVSLIQDVERILDYSLCQETWSKIRAGLPISPVDLSYLAPKNPGTGPAFTIINGTLKYFETRYIRYDIAAPILSRMVGMISGTSTERELWDDWA

SEQ ID NO: 178 - protein, 361 aa, synthetic construct
KFTIVFPHNQKGNWKNVPSNYHYCPSSSDLNWHNDLIGTALQVKMPKSHKAIQADGWMCHASKWVTTCDFRWYGPKYITHSIRSFTPSVEQCKESIEQTKQGTWLNPGFPPQSCGYATVTDAEAVIVQVTPHHVLVDEYTGEWVDSQFINGKCSNYICPTVHNSTTWHSDYKVKGLCDSNLISMDITFFSEDGELSSLGKEGTGFRSNYFAYETGGKACKMQYCKHWGVRLPSGVWFEMADKDLFAAARFPECPEGSSISAPSQTSVDVSLIQDVERILDYSLCQETWSKIRAGLPISPVDLSYLAPKNPGTGPAFTIINGTLKYFETRYERVDIAAPILSRMVGMISGTTTKRELWDDWA

SEQ ID NO: 179 - protein, 361 aa, synthetic construct
KFTIVFPHNVKGNWKNVPSNYHYCPSSSDLNWHNDLIGTALQVKMPKSHHAIQADGWMCHASKWVTTCDFRWYGPKYITHSIRSFTPSVEQCKESIEQTKQGTWLNPGFPPQSCGYATVTDAEAVIVQVTPHHVLVDEYTGEWVDSQFINGKCSNYICPTVHNSTTWHSDYKVKGLCDSNLISMDITFFSEDGELSSLGKEGTGFRSNYFAYETGGKACKMQYCKHWGVRLPSGVWFEMADKDLFAAARFPECPEGSSISAPSQTSVDVSLIQDVERILDYSLCQETWSKIRAGLPISPVDLSYLAPKNPGTGPAFTIINGTLKYFETRYMRVDIAAPILSRMVGMISGTTDERELWDDWA

SEQ ID NO: 180 - protein, 361 aa, synthetic construct
KFTIVFPHAQKGNWKNVPSNYHYCPSSSDLNWHNDLIGTALQVKMPKSHKAIQADGWMCHASKWVTTCDFRWYGPKYITHSIRSFTPSVEQCKESIEQTKQGTWLNPGFPPQSCGYATVTDAEAVIVQVTPHHVLVDEYTGEWVDSQFINGKCSNYICPTVHNSTTWHSDYKVKGLCDSNLISMDITFFSEDGELSSLGKEGTGFRSNYFAYETGGKACKMQYCKHWGVRLPSGVWFEMADKDLFAAARFPECPEGSSISAPSQTSVDVSLIQDVERILDYSLCQETWSKIRAGLPISPVDLSYLAPKNPGTGPAFTIINGTLKYFETRYERVDIAAPILSRMVGMISGTTTSRELWDDWA

SEQ ID NO: 181 - protein, 361 aa, synthetic construct
KFTIVFPGNQKGNWKNVPSNYHYCPSSSDLNWHNDLIGTALQVKMPKSHKSIQADGWMCHASKWVTTCDFRWYGPKYITHSIRSFTPSVEQCKESIEQTKQGTWLNPGFPPQSCGYATVTDAEAVIVQVTPHHVLVDEYTGEWVDSQFINGKCSNYICPTVHNSTTWHSDYKVKGLCDSNLISMDITFFSEDGELSSLGKEGTGFRSNYFAYETGGKACKMQYCKHWGVRLPSGVWFEMADKDLFAAARFPECPEGSSISAPSQTSVDVSLIQDVERILDYSLCQETWSKIRAGLPISPVDLSYLAPKNPGTGPAFTIINGTLKYFETRYIRVDIAAPILSRMVGMISGTTTERWLWDDWA

SEQ ID NO: 182 - protein, 361 aa, synthetic construct
KFTIVFPVNQKGNWKNVPSNYHYCPSSSDLNWHNDLIGTALQVKMPWSHKAIQADGWMCHASKWVTTCDFRWYGPKYITHSIRSFTPSVEQCKESIEQTKQGTWLNPGFPPQSCGYATVTDAEAVIVQVTPHHVLVDEYTGEWVDSQFINGKCSNYICPTVHNSTTWHSDYKVKGLCDSNLISMDITFFSEDGELSSLGKEGTGFRSNYFAYETGGKACKMQYCKHWGVRLPSGVWFEMADKDLFAAARFPECPEGSSISAPSQTSVDVSLIQDVERILDYSLCQETWSKIRAGLPISPVDLSYLAPKNPGTGPAFTIINGTLKYFETRMIRVDIAAPILSRMVGMISGTDTERELWDDWA

SEQ ID NO: 183 - protein, 361 aa, synthetic construct
KFTIVFPHQQKGNWKNVPSNYHYCPSSSDLNWHNDLIGTALQVKMPKSHKPIQADGWMCHASKWVTTCDFRWYGPKYITHSIRSFTPSVEQCKESIEQTKQGTWLNPGFPPQSCGYATVTDAEAVIVQVTPHHVLVDEYTGEWVDSQFINGKCSNYICPTVHNSTTWHSDYKVKGLCDSNLISMDITFFSEDGELSSLGKEGTGFRSNYFAYETGGKACKMQYCKHWGVRLPSGVWFEMADKDLFAAARFPECPEGSSISAPSQTSVDVSLIQDVERILDYSLCQETWSKIRAGLPISPVDLSYLAPKNPGTGPAFTIINGTLKYFETVYIRVDIAAPILSRMVGMISGTTTKRELWDDWA

SEQ ID NO: 184 - protein, 441 aa, synthetic construct
METDTLLLWVLLLWVPGSTGDDCGLPPDVPNAQPALEGRTSFPEDTVITYKCEESFVKIPGEKDSVICLKGSQWSDIEEFCNRSCEVPTRLNSASLKQPYITQNYFPVGTVVEYECRPGYRREPSLSPKLTCLQNLKWSTAVEFCKKKSCPNPGEIRNGQIDVPGGILFGATISFSCNTGYKLFGSTSSFCLISGSSVQWSDPLPECREIYCPAHLQIDNGIIQGERDHYGYRQSVTYACNKGFTMIGEHSIYCTVNNDEGEWSGHLHECRGKSLTSKVPPTVQKPTTVNVPTTEVSPTSQKTTTKTTTPNAQATRSTPVSRTTKHFHETTPNKGSGTTSGGGAHHHHHHFEHPHIQDAASQLPDDESLFFGDTGLSKNPIELVEGWFSSWKSSIASFFFIIGLIIGLFLVLRVGIHLCIKLKHTKKRQIYTDIEMNRLGK

SEQ ID NO: 185 - protein, 379 aa, synthetic construct
METDTLLLWVLLLWVPGSTGDDCGLPPDVPNAQPALEGRTSFPEDTVITYKCEESFVKIPGEKDSVICLKGSQWSDIEEFCNRSCEVPTRLNSASLKQPYITQNYFPVGTVVEYECRPGYRREPSLSPKLTCLQNLKWSTAVEFCKKKSCPNPGEIRNGQIDVPGGILFGATISFSCNTGYKLFGSTSSFCLISGSSVQWSDPLPECREIYCPAHLQIDNGIIQGERDHYGYRQSVTYACNKGFTMIGEHSIYCTVNNDEGEWSGHLHECRGKSLTSKVPPTVQKPTTVNVPTTEVSPTSQKTTTKTTTPNAQATRSTPVSRTTKHFHETTPNKGSGTTSGGGAHHHHHHSGTTRLLSGHTCFTLTGLLGTLVTMGLLT

SEQ ID NO: 186 - protein, 368 aa, synthetic construct
METDTLLLWVLLLWVPGSTGDEDCNELPPRRNTEILTGSWSDQTYPEGTQAIYKCRPGYRSLGNVIMVCRKGEWVALNPLRKCQKRPCGHPGDTPFGTFTLTGGNVFEYGVKAVYTCNEGYQLLGEINYRECDTDGWTNDIPICEVVKCLPVTAPENGKIVSSAMEPDREYHFGQAVRFVCNSGYKIEGDEEMHCSDDGFWSKEKPKCVEISCKSPDVINGSPISQKIIYKENERFQYKCNMGYEYSERGDAVCTESGWRPLPSCEEKGGAHHHHHHFEHPHIQDAASQLPDDESLFFGDTGLSKNPIELVEGWFSSWKSSIASFFFIIGLIIGLFLVLRVGIHLCIKLKHTKKRQIYTDIEMNRLGK

SEQ ID NO: 187 - protein, 306 aa, synthetic construct
METDTLLLWVLLLWVPGSTGDEDCNELPPRRNTEILTGSWSDQTYPEGTQAIYKCRPGYRSLGNVIMVCRKGEWVALNPLRKCQKRPCGHPGDTPFGTFTLTGGNVFEYGVKAVYTCNEGYQLLGEINYRECDTDGWTNDIPICEVVKCLPVTAPENGKIVSSAMEPDREYHFGQAVRFVCNSGYKIEGDEEMHCSDDGFWSKEKPKCVEISCKSPDVINGSPISQKIIYKENERFQYKCNMGYEYSERGDAVCTESGWRPLPSCEEKGGAHHHHHHSGTTRLLSGHTCFTLTGLLGTLVTMGLLT

SEQ ID NO: 188 - protein, 370 aa, synthetic construct
METDTLLLWVLLLWVPGSTGDQDNEKCSQKTLIGYRLKMSRDGDIAVGETVELRCRSGYTTYARNITATCLQGGTWSEPTATCNKKSCPNPGEIQNGKVIFHGGQDALKYGANISYVCNEGYFLVGREYVRYCMIGASGQMAWSSSPPFCEKEKCHRPKIENGDFKPDKDYYEYNDAVHFECNEGYTLVGPHSIACAVNNTWTSNMPTCELAGCKFPSVTHGYPIQGFSLTYKHKQSVTFACNDGFVLRGSPTITCNVTEWDPPLPKCVLGGAHHHHHHFEHPHIQDAASQLPDDESLFFGDTGLSKNPIELVEGWFSSWKSSIASFFFIIGLIIGLFLVLRVGIHLCIKLKHTKKRQIYTDIEMNRLGK

SEQ ID NO: 189 - protein, 308 aa, synthetic construct
METDTLLLWVLLLWVPGSTGDQDNEKCSQKTLIGYRLKMSRDGDIAVGETVELRCRSGYTTYARNITATCLQGGTWSEPTATCNKKSCPNPGEIQNGKVIFHGGQDALKYGANISYVCNEGYFLVGREYVRYCMIGASGQMAWSSSPPFCEKEKCHRPKIENGDFKPDKDYYEYNDAVHFECNEGYTLVGPHSIACAVNNTWTSNMPTCELAGCKFPSVTHGYPIQGFSLTYKHKQSVTFACNDGFVLRGSPTITCNVTEWDPPLPKCVLGGAHHHHHHSGTTRLLSGHTCFTLTGLLGTLVTMGLLT

SEQ ID NO: 190 - protein, 365 aa, synthetic construct
METDTLLLWVLLLWVPGSTGDCCTIPSRPINMTFKNSVETDANANYNIGDTIEYLCLPGYRKQKMGPIYAKCTGTGWTLFNQCIKRRCPSPRDIDNGHLDIGGVDFGSSITYSCNSGYYLIGEYKSYCKLGSTGSMVWNPKAPICESVKCQLPPSISNGRHNGYNDFYTDGSVVTYSCNSGYSLIGNSGVLCSGGEWSNPPTCQIVKCPHPTILNGYLSSGFKRSYSYNDNVDFTCKYGYKLSGSSSSTCSPGNTWQPELPKCVRGGAHHHHHHFEHPHIQDAASQLPDDESLFFGDTGLSKNPIELVEGWFSSWKSSIASFFFIIGLIIGLFLVLRVGIHLCIKLKHTKKRQIYTDIEMNRLGK

SEQ ID NO: 191 - protein, 303 aa, synthetic construct
METDTLLLWVLLLWVPGSTGDCCTIPSRPINMTFKNSVETDANANYNIGDTIEYLCLPGYRKQKMGPIYAKCTGTGWTLFNQCIKRRCPSPRDIDNGHLDIGGVDFGSSITYSCNSGYYLIGEYKSYCKLGSTGSMVWNPKAPICESVKCQLPPSISNGRHNGYNDFYTDGSVVTYSCNSGYSLIGNSGVLCSGGEWSNPPTCQIVKCPHPTILNGYLSSGFKRSYSYNDNVDFTCKYGYKLSGSSSSTCSPGNTWQPELPKCVRGGAHHHHHHSGTTRLLSGHTCFTLTGLLGTLVTMGLLT

SEQ ID NO: 192 - protein, 184 aa, synthetic construct
METDTLLLWVLLLWVPGSTGDGHSLQAAQHDEAVDANSLAEAKVLANRELDKYGVSDYYKNLINNAKTVEGVKALIDEILAALPGGAHHHHHHFEHPHIQDAASQLPDDESLFFGDTGLSKNPIELVEGWFSSWKSSIASFFFIIGLIIGLFLVLRVGIHLCIKLKHTKKRQIYTDIEMNRLGK

SEQ ID NO: 193 - protein, 123 aa, synthetic construct
METDTLLLWVLLLWVPGSTGDGHSLQAAQHDEAVDANSLAEAKVLANRELDKYGVSDYYKNLINNAKTVEGVKALIDEILAALPGGAHHHHHHNLENGGTSLSEKTVLLLVTPFLAAAWSLHP

SEQ ID NO: 194 - DNA, 690 bp, synthetic construct
  source 1..690: mol_type = other DNA
agctagagattctgggggcccttcaaacttctttgggacatgtatgtgtaatttcctagtaaaagagttttgcctgcttcttcttctttctccccctggtgtctgcctgcagtactacaatctccctagtggtgaaatagtgtgcctgcctttgttctccgaggctcacaacatgctattcaactctgcactctgagtcaggcaagacagaaaccagtaccttgggtaacccccacaaaacccaggagaaacagtttgagagagggcagtggagaagcaagagagctggtctggaacccagctgcctgactcgtgagtcatttctcttcctccaaagccctattaagtctggggctgcttatggtcctcaccaactacacaaagaaagtcagggtcatgctcatccatcaggaggttcagggccacttcccgctttcctctgtttggcaacactaagagtcaccctctgattgttccagaaaagcaagaattgctaaaggccattgtgtcaagtttgcccaattcatgctgcttgacatcttacccctccccaccctgctcccatcccccccacccagtgcccctgattgcaacactcctggctggggtgggacagggtggccagataaaagcagagcaggacctggaaagctggtttgtatgggctgcagcctgccgctgagctgcatc

SEQ ID NO: 195 - protein, 491 aa, synthetic construct
MGQIVTFFQEVPHVIEEVMNIVLIALSVLAVLKGLYNFATCGLVGLVTFLLLCGRSCTTSLYKGVYELQTLELNMETLNMTMPLSCTKNNSHHYIMVGNETGLELTLTNTSIINHKFCNLSDAHKKNLYDHALMSIISTFALSIPNANQYEAMSCDFNGGKISVQYNLSHSYAGDAANHCGTVANGVLQTFMRMAWGGSYIALDSGRGNWDCIMTSYQYLIIQNTTWEDHCQFSRPSPIGYLGLLSQRTRDIYISRRLLGTFTWTLSDSEGKDTPGGYCLTRWMLIEAELKCFGNTAVAKCNEKHDEEFCDMLRLFDFNKQAIQRLKAEAQMSIQLINKAVNALINDQLIMKNHLRDIMGIPYCNYSKYWYLNHTTTGRTSLPKCWLVSNGSYLNETHFSDDIEQQADNMITEMLQKEYMERQGKTPLGLVDLFVFSTSFYLISIFLHLVKIPTHRHIVGKSCPKPHRLNHMGICSCGLYKQPGVPVKWKR

SEQ ID NO: 196 - protein, 491 aa, synthetic construct
MGQIVTFFQEVPHVIEEVMNIVLIALSVLAVLKGLYNFATCGLVGLVTFLLLCGRSCTTSLYKGVYELQTLELNMETLNMTMPLSCTKNNSHHYIMVGNETGLELTLTNTSIINHKFCNLSDAHKKNLYDHALMSIISTFHLSIPNFNQYEAMSCDFNGGKISVQYNLSHSYAGDAANHCGTVANGVLQTFMRMAWGGSYIALDSGRGNWDCIMTSYQYLIIQNTTWEDHCQFSRPSPIGYLGLLSQRTRDIYISRRLLGTFTWTLSDSEGKDTPGGYCLTRWMLIEAELKCFGNTAVAKCNEKHDEEFCDMLRLFDFNKQAIQRLKAEAQMSIQLINKAVNALINDQLIMKNHLRDIMGIPYCNYSKYWYLNHTTTGRTSLPKCWLVSNGSYLNETHFSDDIEQQADNMITEMLQKEYMERQGKTPLGLVDLFVFSTSFYLISILLHLVKIPTHRHIVGKSCPKPHRLNHMGICSCGLYKQPGVPVKWKR

SEQ ID NO: 197 - protein, 491 aa, synthetic construct
MGQIVTFFQEVPHVIEEVMNIVLIALSVLAVLKGLYNFATCGLVGLVTFLLLCGRSCTTSLYKGVYELQTLELNMETLNMTMPLSCTKNNSHHYIMVGNETGLELTLTNTSIINHKFCNLSDAHKKNLYDHALMSIISTFHLSIPNFNQYEAMSCDFNGGKISVQYNLSHSYAGDAANHCGTVANGVLQTFMRMAWGGSYIALDSGRGNWDCIMTSYQYLIIQNTTWEDHCQFSRPSPIGYLGLLSQRTRDIYISRRLLGTFTWTLSDSEGKDTPGGYCLTRWMLIEAELKCFGNTAVAKCNEKHDEEFCDMLRLFDFNKQAIQRLKAEAQMSIQLINKAVNALINDQLIMKNHLRDIMGIPYCNYSKYWYLNHTTTGRTSLPKCWLVSNGSYLNETHFSDDIEQQADNMITEMLQKEYMERQGKTPLGLVDLFVFSTSFYLISIFLHLVKIPTHRHIVGKSCPKPHRLNHMGICSCGLYKQPGVPVKWKR

SEQ ID NO: 198 - DNA, 445 bp, synthetic construct
  source 1..445: mol_type = other DNA
gagaaacagtttgagagagggcagtggagaagcaagagagctggtctggaacccagctgcctgactcgtgagtcatttctcttcctccaaagccctattaagtctggggctgcttatggtcctcaccaactacacaaagaaagtcagggtcatgctcatccatcaggaggttcagggccacttcccgctttcctctgtttggcaacactaagagtcaccctctgattgttccagaaaagcaagaattgctaaaggccattgtgtcaagtttgcccaattcatgctgcttgacatcttacccctccccaccctgctcccatcccccccacccagtgcccctgattgcaacactcctggctggggtgggacagggtggccagataaaagcagagcaggacctggaaagctggtttgtatgggctgcagcctgccgctgagctgcatc

SEQ ID NO: 199 - protein, 273 aa, synthetic construct
MGHTRRQGTSPSKCPYLNFFQLLVLAGLSHFCSGVIHVTKEVKEVATLSCGHNVSVEELAQTRIYWQKEKKMVLTMMSGDMNIWPEYKNRTIFDITNNLSIVILALRPSDEGTYECVVLKYEKDAFKREHLAEVTLSVKADFPTPSISDFEIPTSNIRRIICSTSGGFPEPHLSWLENGEELNAINTTVSQDPETELYAVSSKLDFNMTTNHSFMCLIKYGHLRVNQTFNWNTTKQEHFPDNLLPSWAITLISVNGIFVICCLTYCFAPRCRE

SEQ ID NO: 200 - protein, 247 aa, synthetic construct
EVKLQQSGPGLVTPSQSLSITCTVSGFSLSDYGVHWVRQSPGQGLEWLGVIWAGGGTNYNSALMSRKSISKDNSKSQVFLKMNSLQADDTAVYYCARDKGYSYYYSMDYWGQGTSVTVSSGGGGSGGGGSGGGGSDIELTQSPASLAVSLGQRATISCRASESVEYYVTSLMQWYQQKPGQPPKLLIFAASNVESGVPARFSGSGSGTNFSLNIHPVDEDDVAMYFCQQSRKVPYTFGGGTKLEIKR

SEQ ID NO: 201 - protein, 64 aa, synthetic construct
GGGGSGGGGSGGGGSAVGQDTQEVIVVPHSLPFKVVVISAILALVVLTIISLIILIMLWQKKPR

SEQ ID NO: 202 - protein, 307 aa, synthetic construct
METDTLLLWVLLLWVPGSTGDQVQLQQPGAELVKPGASVKLSCKASGYTFSSYWMHWVKQRPGQVLEWIGEINPGNGHTNYNEKFKSKATLTVDKSSSTAYMQLSSLTSEDSAVYYCARSFTTARGFAYWGQGTLVTVSAGGGGSGGGGSGGGGSDIVMTQSPATQSVTPGDRVSLSCRASQTISDYLHWYQQKSHESPRLLIKYASQSISGIPSRFSGSGSGSDFTLSINSVEPEDVGVYYCQDGHSFPPTFGGGTKLEIKSASESKYGPPCPPCPVVVISAILALVVLTIISLIILIMLWQKKPR

SEQ ID NO: 203 - protein, 511 aa, unidentified
MKCLLYLAFLFIGVNCKFTIVFPHNQKGNWKNVPSNYHYCPSSSDLNWHNDLIGTAIQVKMPKSHKAIQADGWMCHASKWVTTCDFRWYGPKYITQSIRSFTPSVEQCKESIEQTKQGTWLNPGFPPQSCGYATVTDAEAVIVQVTPHHVLVDEYTGEWVDSQFINGKCSNYICPTVHNSTTWHSDYKVKGLCDSNLISMDITFFSEDGELSSLGKEGTGFRSNYFAYETGGKACKMQYCKHWGVRLPSGVWFEMADKDLFAAARFPECPEGSSISAPSQTSVDVSLIQDVERILDYSLCQETWSKIRAGLPISPVDLSYLAPKNPGTGPAFTIINGTLKYFETRYIRVDIAAPILSRMVGMISGTTTERELWDDWAPYEDVEIGPNGVLRTSSGYKFPLYMIGHGMLDSDLHLSSKAQVFEHPHIQDAASQLPDDESLFFGDTGLSKNPIELVEGWFSSWKSSIASFFFIIGLIIGLFLVLRVGIHLCIKLKHTKKRQIYTDIEMNRLGK

SEQ ID NO: 204 - protein, 495 aa, unidentified
KFTIVFPHNQKGNWKNVPSNYHYCPSSSDLNWHNDLIGTAIQVKMPKSHKAIQADGWMCHASKWVTTCDFRWYGPKYITQSIRSFTPSVEQCKESIEQTKQGTWLNPGFPPQSCGYATVTDAEAVIVQVTPHHVLVDEYTGEWVDSQFINGKCSNYICPTVHNSTTWHSDYKVKGLCDSNLISMDITFFSEDGELSSLGKEGTGFRSNYFAYETGGKACKMQYCKHWGVRLPSGVWFEMADKDLFAAARFPECPEGSSISAPSQTSVDVSLIQDVERILDYSLCQETWSKIRAGLPISPVDLSYLAPKNPGTGPAFTIINGTLKYFETRYIRVDIAAPILSRMVGMISGTTTERELWDDWAPYEDVEIGPNGVLRTSSGYKFPLYMIGHGMLDSDLHLSSKAQVFEHPHIQDAASQLPDDESLFFGDTGLSKNPIELVEGWFSSWKSSIASFFFIIGLIIGLFLVLRVGIHLCIKLKHTKKRQIYTDIEMNRLGK